European Patent Application EP 4 385 567 A2, published June 19, 2024. Title: METHODS AND COMPOSITIONS FOR RNA-GUIDED TREATMENT OF HIV INFECTION. Applicant: TEMPLE UNIVERSITY OF THE COMMONWEALTH SYSTEM OF HIGHER EDUCATION. The sequence listing filed with the application follows.

SEQUENCE LISTING (389 sequences)

SEQ ID NO: 1 - DNA, 30 bp, Human immunodeficiency virus 1
  source 1..30: mol_type = unassigned DNA
gccagggatcagatatccactgacctttgg

SEQ ID NO: 2 - DNA, 34 bp, Human immunodeficiency virus 1
  source 1..34: mol_type = unassigned DNA
tccggagtacttcaagaactgctgacatcgagct

SEQ ID NO: 3 - DNA, 19 bp, synthetic construct
  misc_feature 1..19: note = Description of Artificial Sequence: Synthetic oligonucleotide
  source 1..19: mol_type = other DNA
ccactgactacttcaagaa

SEQ ID NO: 4 - DNA, 859 bp, synthetic construct
  modified_base 289..313: mod_base = OTHER; note = a, c, t, or g
  source 1..859: mol_type = other DNA
ctaggtgattaggatattctacaatccaaattcttaccagtttgggattattcaaattgggcaccttggcagatatgttttgaaaactgctaggcaaagcattctggaagaatagacaaagaagtaataaaatataacaaaaagcagtggaagttacaaaaaaaaatgtttctcttttggaagggctaatttggtcccaaagaagacaagatatccttgatctgtggatctaccacacacaaggctacttccctgattggcagaactacaacaccagggccagggatcnnnnnnnnnnnnnnnnnnnnnnnnnttcaagttagtaccagttgagccagggcaggtagaagaggccaatgaaggagagaacaacaccttgttacaccctatgagcctgcatgggatggaggacccggagggagaagtattagtgtggaagtttgacagcctcctagcatttcgtcacatggcccgagagctgcatccggagtactacaaagactgctgacatcgagttttctacaagggactttccgctggggactttccagggaggtgtggcctgggcgggactggggagtggcgagccctcagatgctgcatataagcagctgctttttgcctgtactgggtctctctggttagaccagatctgagcctgggagctctctggctagctagggaacccactgcttaagcctcaataaagcttgccttgagtgctacaagtagtgtgtgcccgtctgttgtgtgactctggtaactagagatccctcagacccttttagtcagtgtggaaaatctctagcatctttaaagtacagaatgccaaaacaggaaggattgataagatagtcgt

SEQ ID NO: 5 - DNA, 10 bp, Human immunodeficiency virus 1
  source 1..10: mol_type = unassigned DNA
tcttttggaa

SEQ ID NO: 6 - DNA, 76 bp, Human immunodeficiency virus 1
  source 1..76: mol_type = unassigned DNA
gattggcagaactacacaccagggccagggatcagatatccactgacctttggatggtgcttcaagttagtaccag

SEQ ID NO: 7 - DNA, 10 bp, Human immunodeficiency virus 1
  source 1..10: mol_type = unassigned DNA
tctttaaagt

SEQ ID NO: 8 - DNA, 10 bp, synthetic construct
  misc_feature 1..10: note = Description of Artificial Sequence: Synthetic oligonucleotide
  source 1..10: mol_type = other DNA
tcttttggaa

SEQ ID NO: 9 - DNA, 63 bp, synthetic construct
  misc_feature 1..63: note = Description of Artificial Sequence: Synthetic oligonucleotide
  source 1..63: mol_type = other DNA
gattggcagaactacaacaccagggccagggatcagatggatggtgcttcaagttagtaccag

SEQ ID NO: 10 - DNA, 10 bp, synthetic construct
  misc_feature 1..10: note = Description of Artificial Sequence: Synthetic oligonucleotide
  source 1..10: mol_type = other DNA
tctttaaagt

SEQ ID NO: 11 - DNA, 10 bp, synthetic construct
  misc_feature 1..10: note = Description of Artificial Sequence: Synthetic oligonucleotide
  source 1..10: mol_type = other DNA
tcttttggaa

SEQ ID NO: 12 - DNA, 50 bp, synthetic construct
  misc_feature 1..50: note = Description of Artificial Sequence: Synthetic oligonucleotide
  source 1..50: mol_type = other DNA
gattggcagaactacaacaccagggccagggatcttcaagttagtaccag

SEQ ID NO: 13 - DNA, 10 bp, synthetic construct
  misc_feature 1..10: note = Description of Artificial Sequence: Synthetic oligonucleotide
  source 1..10: mol_type = other DNA
tctttaaagt

SEQ ID NO: 14 - DNA, 24 bp, synthetic construct
  misc_feature 1..24: note = Description of Artificial Sequence: Synthetic oligonucleotide
  source 1..24: mol_type = other DNA
gagatcctgtctcaaaaaaaagtt

SEQ ID NO: 15 - DNA, 17 bp, synthetic construct
  misc_feature 1..17: note = Description of Artificial Sequence: Synthetic oligonucleotide
  source 1..17: mol_type = other DNA
atctatccatgagggcg

SEQ ID NO: 16 - DNA, 402 bp, Human immunodeficiency virus 1
  source 1..402: mol_type = unassigned DNA
gatctgtggatctaccacacacaaggctacttccctgattggcagaactacacaccagggccagggatcagatatccactgacctttggatggtgctacaagctagtaccagttgagcaagagaaggtagaagaagccaatgaaggagagaacacccgcttgttacaccctgtgagcctgcatgggatggatgacccggagagagaagtattagagtggaggtttgacagccgcctagcatttcatcacatggcccgagagctgcatccggagtacttcaagaactgctgacatcgagcttgctacaagggactttccgctggggactttccagggaggcgtggcctgggcgggactggggagtggcgagccctcagatgctgcatataagcagctgctttt

SEQ ID NO: 17 - DNA, 31 bp, Human immunodeficiency virus 1
  source 1..31: mol_type = unassigned DNA
ccctgattggcagaactacacaccagggcca

SEQ ID NO: 18 - DNA, 32 bp, synthetic construct
  misc_feature 1..32: note = Description of Artificial Sequence: Synthetic oligonucleotide
  source 1..32: mol_type = other DNA
ccctgattggcagaactacaacaccagggcca

SEQ ID NO: 19 - DNA, 32 bp, synthetic construct; identical to SEQ ID NO: 18
  misc_feature 1..32: note = Description of Artificial Sequence: Synthetic oligonucleotide
  source 1..32: mol_type = other DNA

SEQ ID NO: 20 - DNA, 32 bp, synthetic construct; identical to SEQ ID NO: 18
  misc_feature 1..32: note = Description of Artificial Sequence: Synthetic oligonucleotide
  source 1..32: mol_type = other DNA

SEQ ID NO: 21 - DNA, 30 bp, synthetic construct
  misc_feature 1..30: note = Description of Artificial Sequence: Synthetic oligonucleotide
  source 1..30: mol_type = other DNA
ccctgattggcagaactacaaccagggcca

SEQ ID NO: 22 - DNA, 29 bp, synthetic construct
  misc_feature 1..29: note = Description of Artificial Sequence: Synthetic oligonucleotide
  source 1..29: mol_type = other DNA
ccctgattggcagaactacaccagggcca

SEQ ID NO: 23 - DNA, 29 bp, synthetic construct
  misc_feature 1..29: note = Description of Artificial Sequence: Synthetic oligonucleotide
  source 1..29: mol_type = other DNA
ccctgattggcagaactacaccagggcca

SEQ ID NO: 24 - DNA, 26 bp, synthetic construct
  misc_feature 1..26: note = Description of Artificial Sequence: Synthetic oligonucleotide
  source 1..26: mol_type = other DNA
ccctgattggcagaactacagggcca

SEQ ID NO: 25 - DNA, 29 bp, synthetic construct
  misc_feature 1..29: note = Description of Artificial Sequence: Synthetic oligonucleotide
  source 1..29: mol_type = other DNA
ccctgattggcagaactacagggccaggg

SEQ ID NO: 26 - DNA, 86 bp, Human immunodeficiency virus 1
  source 1..86: mol_type = unassigned DNA
gactttccagggaggcgtggcctgggcgggactggggagtggcgagccctcagatgctgcatataagcagcggtgaagccgaattc

SEQ ID NO: 27 - DNA, 86 bp, synthetic construct
  misc_feature 1..86: note = Description of Artificial Sequence: Synthetic oligonucleotide
  source 1..86: mol_type = other DNA
gactttccagggaggcgtggcctgggcgggactggggggtggcgagccctcagatgctgcatataagcagcggtgaagccgaattc

SEQ ID NO: 28 - DNA, 88 bp, synthetic construct
  misc_feature 1..88: note = Description of Artificial Sequence: Synthetic oligonucleotide
  source 1..88: mol_type = other DNA
gactttccagggaggcgtggcctgggcgggtatctggggagtggcgagccctcagatgctgcatataagcagcggtgaagccgaattc

SEQ ID NO: 29 - DNA, 85 bp, synthetic construct
  misc_feature 1..85: note = Description of Artificial Sequence: Synthetic oligonucleotide
  source 1..85: mol_type = other DNA
gactttccaggggggcgtggcctgggcgggactggggagtggcgagccctcagatgctgcataaagcagcggtgaagccgaattc

SEQ ID NO: 30 - DNA, 23 bp, synthetic construct
  misc_feature 1..23: note = Description of Artificial Sequence: Synthetic oligonucleotide
  source 1..23: mol_type = other DNA
gactttccagggaagccgaattc

SEQ ID NO: 31 - DNA, 25 bp, synthetic construct
  misc_feature 1..25: note = Description of Artificial Sequence: Synthetic oligonucleotide
  source 1..25: mol_type = other DNA
gattggcagaactacactggggagt

SEQ ID NO: 32 - DNA, 26 bp, synthetic construct
  misc_feature 1..26: note = Description of Artificial Sequence: Synthetic oligonucleotide
  source 1..26: mol_type = other DNA
gattggcagaactacacctcagatgc

SEQ ID NO: 33 - DNA, 28 bp, synthetic construct
  misc_feature 1..28: note = Description of Artificial Sequence: Synthetic oligonucleotide
  source 1..28: mol_type = other DNA
catcacatggcccgctgctgacatcgag

SEQ ID NO: 34 - DNA, 55 bp, Human immunodeficiency virus 1
  source 1..55: mol_type = unassigned DNA
catcacgtggcccgagagctgcatccggagtacttcaagaactgctgacatcgag

SEQ ID NO: 35 - DNA, 1106 bp, synthetic construct
  modified_base 152..155: mod_base = OTHER; note = a, c, t, or g
  source 1..1106: mol_type = other DNA
gctattgtatctgatcacaagctgttaaaagcggtcatgccacttcttgaatgctttgcagctggaagggctaatttggtcccaaagaagacaagatatccttgatctgtggatctaccacacacaaggctacttccctgattggcagaacnnnncaccagggccagggatcagatatccactgaccatccactttggatggtgcttcaagttagtaccagttgagccagggcaggtagaagaggccaatgaaggagagaacaacaccttgttacaccctatgagcctgcatgggatggaggacccggagggagaagtattagtgtggaagtttgacagcctcctagcatttcgtcacatggcccgagagctgcatccggagtactacaaagactgctgacatcgagttttctacaagggactttccgctggggactttccagggaggtgtggcctgggcgggactggggagtggcgagccctcagatgctgcatataagcagctgctttttgcctgtactgggtctctctggttagaccagatctgagcctgggagctctctggctagctagggaacccactgcttaagcctcaataaagcttgccttgagtgctacaagtagtgtgtgcccgtctgttgtgtgactctggtaactagagatccctcagacccttttagtcagtgtggaaaatctctagcagcagcttagaaattttttccaccagaggccgggcgtggtggctcacgcctgtaatcccagcactttgggaggccgaggtgggcggatcacctgaagtcaggagttcgagaccagcctcaacatggagaaaccccatctctactaaaaatacaaaattagctgggcgtggtggtgcatgcctgtaatcccagctacttgggaggctgagacaggataattgcttgaacctggaaggcagaggttgcggtgagccgagattgcgccattgcattccagcctgggcaacaggagcgaaacttcgtctcaaaaaaaaaaaaaaaagacattttttccaccagataccctagatcatgactgttaagtctggccttccacgaagccctaggacctggacacacaatcaa

SEQ ID NO: 36 - DNA, 36 bp, synthetic construct
  misc_feature 1..36: note = Description of Artificial Sequence: Synthetic oligonucleotide
  source 1..36: mol_type = other DNA
aaacagggccagggatcagatatccactgaccttgt

SEQ ID NO: 37 - DNA, 35 bp, synthetic construct
  misc_feature 1..35: note = Description of Artificial Sequence: Synthetic oligonucleotide
  source 1..35: mol_type = other DNA
taaacaaggtcagtggatatctgatccctggccct

SEQ ID NO: 38 - DNA, 36 bp, synthetic construct
  misc_feature 1..36: note = Description of Artificial Sequence: Synthetic oligonucleotide
  source 1..36: mol_type = other DNA
aaacagctcgatgtcagcagttcttgaagtactcgt

SEQ ID NO: 39 - DNA, 35 bp, synthetic construct
  misc_feature 1..35: note = Description of Artificial Sequence: Synthetic oligonucleotide
  source 1..35: mol_type = other DNA
taaacgagtacttcaagaactgctgacatcgagct

SEQ ID NO: 40 - DNA, 24 bp, synthetic construct
  misc_feature 1..24: note = Description of Artificial Sequence: Synthetic oligonucleotide
  source 1..24: mol_type = other DNA
caccgattggcagaactacacacc

SEQ ID NO: 41 - DNA, 24 bp, synthetic construct
  misc_feature 1..24: note = Description of Artificial Sequence: Synthetic oligonucleotide
  source 1..24: mol_type = other DNA
aaacggtgtgtagttctgccaatc

SEQ ID NO: 42 - DNA, 24 bp, synthetic construct
  misc_feature 1..24: note = Description of Artificial Sequence: Synthetic oligonucleotide
  source 1..24: mol_type = other DNA
caccgcgtggcctgggcgggactg

SEQ ID NO: 43 - DNA, 24 bp, synthetic construct
  misc_feature 1..24: note = Description of Artificial Sequence: Synthetic oligonucleotide
  source 1..24: mol_type = other DNA
aaaccagtcccgcccaggccacgc

SEQ ID NO: 44 - DNA, 24 bp, synthetic construct
  misc_feature 1..24: note = Description of Artificial Sequence: Synthetic primer
  source 1..24: mol_type = other DNA
tggaagggctaattcactcccaac

SEQ ID NO: 45 - DNA, 24 bp, synthetic construct
  misc_feature 1..24: note = Description of Artificial Sequence: Synthetic primer
  source 1..24: mol_type = other DNA
ccgagagctcccaggctcagatct

SEQ ID NO: 46 - DNA, 27 bp, synthetic construct
  misc_feature 1..27: note = Description of Artificial Sequence: Synthetic primer
  source 1..27: mol_type = other DNA
caccgatctgtggatctaccacacaca

SEQ ID NO: 47 - DNA, 24 bp, synthetic construct
  misc_feature 1..24: note = Description of Artificial Sequence: Synthetic primer
  source 1..24: mol_type = other DNA
aaacgagtcacacaacagacgggc

SEQ ID NO: 48 - DNA, 37 bp, synthetic construct
  misc_feature 1..37: note = Description of Artificial Sequence: Synthetic primer
  source 1..37: mol_type = other DNA
cgcctcgaggatccgagggcctatttcccatgattcc

SEQ ID NO: 49 - DNA, 35 bp, synthetic construct
  misc_feature 1..35: note = Description of Artificial Sequence: Synthetic primer
  source 1..35: mol_type = other DNA
tgtgaattcaggcgggccatttaccgtaagttatg

SEQ ID NO: 50 - DNA, 25 bp, synthetic construct
  misc_feature 1..25: note = Description of Artificial Sequence: Synthetic primer
  source 1..25: mol_type = other DNA
acgactatcttatcaatccttcctg

SEQ ID NO: 51 - DNA, 26 bp, synthetic construct
  misc_feature 1..26: note = Description of Artificial Sequence: Synthetic primer
  source 1..26: mol_type = other DNA
ctaggtgattaggatattctacaatc

SEQ ID NO: 52 - DNA, 24 bp, synthetic construct
  misc_feature 1..24: note = Description of Artificial Sequence: Synthetic primer
  source 1..24: mol_type = other DNA
gctattgtatctgatcacaagctg

SEQ ID NO: 53 - DNA, 24 bp, synthetic construct
  misc_feature 1..24: note = Description of Artificial Sequence: Synthetic primer
  source 1..24: mol_type = other DNA
ttgattgtgtgtccaggtcctagg

SEQ ID NO: 54 - DNA, 23 bp, synthetic construct
  misc_feature 1..23: note = Description of Artificial Sequence: Synthetic primer
  source 1..23: mol_type = other DNA
gcaagggcgaggagctgttcacc

SEQ ID NO: 55 - DNA, 24 bp, synthetic construct
  misc_feature 1..24: note = Description of Artificial Sequence: Synthetic primer
  source 1..24: mol_type = other DNA
ttgtagttgccgtcgtccttgaag

SEQ ID NO: 56 - DNA, 23 bp, synthetic construct
  misc_feature 1..23: note = Description of Artificial Sequence: Synthetic primer
  source 1..23: mol_type = other DNA
aatggtacatcaggccatatcac

SEQ ID NO: 57 - DNA, 23 bp, synthetic construct
  misc_feature 1..23: note = Description of Artificial Sequence: Synthetic primer
  source 1..23: mol_type = other DNA
cccactgtgtttagcatggtatt

SEQ ID NO: 58 - DNA, 23 bp, synthetic construct
  misc_feature 1..23: note = Description of Artificial Sequence: Synthetic primer
  source 1..23: mol_type = other DNA
cacagcatcaagaagaacctgat

SEQ ID NO: 59 - DNA, 24 bp, synthetic construct
  misc_feature 1..24: note = Description of Artificial Sequence: Synthetic primer
  source 1..24: mol_type = other DNA
tcttccgtctggtgtatcttcttc

SEQ ID NO: 60 - DNA, 28 bp, synthetic construct
  misc_feature 1..28: note = Description of Artificial Sequence: Synthetic primer
  source 1..28: mol_type = other DNA
cgccaagcttgaataggagctttgttcc

SEQ ID NO: 61 - DNA, 30 bp, synthetic construct
  misc_feature 1..30: note = Description of Artificial Sequence: Synthetic primer
  source 1..30: mol_type = other DNA
ctaggatccaggagctgttgatcctttagg

SEQ ID NO: 62 - DNA, 23 bp, synthetic construct
  misc_feature 1..23: note = Description of Artificial Sequence: Synthetic oligonucleotide
  source 1..23: mol_type = other DNA
gtggactttggatggtgagatag

SEQ ID NO: 63 - DNA, 23 bp, synthetic construct
  misc_feature 1..23: note = Description of Artificial Sequence: Synthetic oligonucleotide
  source 1..23: mol_type = other DNA
gcctggcaagagtgaactgagtc

SEQ ID NO: 64 - DNA, 23 bp, synthetic construct
  misc_feature 1..23: note = Description of Artificial Sequence: Synthetic oligonucleotide
  source 1..23: mol_type = other DNA
aagataatgagttgtggcagagc

SEQ ID NO: 65 - DNA, 24 bp, synthetic construct
  misc_feature 1..24: note = Description of Artificial Sequence: Synthetic oligonucleotide
  source 1..24: mol_type = other DNA
tctacctggtaatccagcatctgg

SEQ ID NO: 66 - DNA, 23 bp, synthetic construct
  misc_feature 1..23: note = Description of Artificial Sequence: Synthetic oligonucleotide
  source 1..23: mol_type = other DNA
ataggaggaaggcaccaagaggg

SEQ ID NO: 67 - DNA, 23 bp, synthetic construct
  misc_feature 1..23: note = Description of Artificial Sequence: Synthetic oligonucleotide
  source 1..23: mol_type = other DNA
aatgatgctttggtcctactcct

SEQ ID NO: 68 - DNA, 24 bp, synthetic construct
  misc_feature 1..24: note = Description of Artificial Sequence: Synthetic oligonucleotide
  source 1..24: mol_type = other DNA
tgctcttgctactctggcatgtac

SEQ ID NO: 69 - DNA, 23 bp, synthetic construct
  misc_feature 1..23: note = Description of Artificial Sequence: Synthetic oligonucleotide
  source 1..23: mol_type = other DNA
aatctacctctgagagctgcagg

SEQ ID NO: 70 - DNA, 23 bp, synthetic construct
  misc_feature 1..23: note = Description of Artificial Sequence: Synthetic oligonucleotide
  source 1..23: mol_type = other DNA
tcagacacagctgaagcagaggc

SEQ ID NO: 71 - DNA, 23 bp, synthetic construct
  misc_feature 1..23: note = Description of Artificial Sequence: Synthetic oligonucleotide
  source 1..23: mol_type = other DNA
atgccagtgtcagtagatgtcag

SEQ ID NO: 72 - DNA, 24 bp, synthetic construct
  misc_feature 1..24: note = Description of Artificial Sequence: Synthetic oligonucleotide
  source 1..24: mol_type = other DNA
tcaagatcagccagagtgcacatg

SEQ ID NO: 73 - DNA, 23 bp, synthetic construct
  misc_feature 1..23: note = Description of Artificial Sequence: Synthetic oligonucleotide
  source 1..23: mol_type = other DNA
tgctcttccgagcctctctggag

SEQ ID NO: 74 - DNA, 22 bp, synthetic construct
  misc_feature 1..22: note = Description of Artificial Sequence: Synthetic oligonucleotide
  source 1..22: mol_type = other DNA
atggactatcatatgcttaccg

SEQ ID NO: 75 - DNA, 28 bp, synthetic construct
  misc_feature 1..28: note = Description of Artificial Sequence: Synthetic oligonucleotide
  source 1..28: mol_type = other DNA
gcttcagcaagccgagtcctgcgtcgag

SEQ ID NO: 76 - DNA, 28 bp, synthetic construct
  misc_feature 1..28: note = Description of Artificial Sequence: Synthetic oligonucleotide
  source 1..28: mol_type = other DNA
gctcctctggtttccctttcgctttcaa

SEQ ID NO: 77 - DNA, 22 bp, synthetic construct
  misc_feature 1..22: note = Description of Artificial Sequence: Synthetic oligonucleotide
  source 1..22: mol_type = other DNA
gtaatacgactcactatagggc

SEQ ID NO: 78 - DNA, 19 bp, synthetic construct
  misc_feature 1..19: note = Description of Artificial Sequence: Synthetic oligonucleotide
  source 1..19: mol_type = other DNA
actatagggcacgcgtggt

SEQ ID NO: 79 - DNA, 23 bp, synthetic construct
  misc_feature 1..23: note = Description of Artificial Sequence: Synthetic oligonucleotide
  source 1..23: mol_type = other DNA
tcagacccttttagtcagtgtgg

SEQ ID NO: 80 - DNA, 23 bp, synthetic construct
  misc_feature 1..23: note = Description of Artificial Sequence: Synthetic oligonucleotide
  source 1..23: mol_type = other DNA
ttgcttgtactgggtctctctgg

SEQ ID NO: 81 - DNA, 23 bp, synthetic construct
  misc_feature 1..23: note = Description of Artificial Sequence: Synthetic oligonucleotide
  source 1..23: mol_type = other DNA
cagctgctttttgcttgtactgg

SEQ ID NO: 82 - DNA, 23 bp, synthetic construct
  misc_feature 1..23: note = Description of Artificial Sequence: Synthetic oligonucleotide
  source 1..23: mol_type = other DNA
ctgacatcgagcttgctacaagg

SEQ ID NO: 83 - DNA, 23 bp, synthetic construct
  misc_feature 1..23: note = Description of Artificial Sequence: Synthetic oligonucleotide
  source 1..23: mol_type = other DNA
ccgcctagcatttcatcacatgg

SEQ ID NO: 84 - DNA, 23 bp, synthetic construct
  misc_feature 1..23: note = Description of Artificial Sequence: Synthetic oligonucleotide
  source 1..23: mol_type = other DNA
cggagagagaagtattagagtgg

SEQ ID NO: 85 - DNA, 23 bp, synthetic construct
  misc_feature 1..23: note = Description of Artificial Sequence: Synthetic oligonucleotide
  source 1..23: mol_type = other DNA
agtaccagttgagcaagagaagg

SEQ ID NO: 86 - DNA, 23 bp, synthetic construct
  misc_feature 1..23: note = Description of Artificial Sequence: Synthetic oligonucleotide
  source 1..23: mol_type = other DNA
gatatccactgacctttggatgg

SEQ ID NO: 87 - DNA, 23 bp, synthetic construct
  misc_feature 1..23: note = Description of Artificial Sequence: Synthetic oligonucleotide
  source 1..23: mol_type = other DNA
gattggcagaactacacaccagg

SEQ ID NO: 88 - DNA, 23 bp, synthetic construct
  misc_feature 1..23: note = Description of Artificial Sequence: Synthetic oligonucleotide
  source 1..23: mol_type = other DNA
cacaaggctacttccctgattgg

SEQ ID NO: 89 - DNA, 23 bp, synthetic construct
  misc_feature 1..23: note = Description of Artificial Sequence: Synthetic oligonucleotide
  source 1..23: mol_type = other DNA
ctgtggatctaccacacacaagg

SEQ ID NO: 90 - DNA, 23 bp, synthetic construct
  misc_feature 1..23: note = Description of Artificial Sequence: Synthetic oligonucleotide
  source 1..23: mol_type = other DNA
tgggagctctctggctaactagg

SEQ ID NO: 91 - DNA, 23 bp, synthetic construct
  misc_feature 1..23: note = Description of Artificial Sequence: Synthetic oligonucleotide
  source 1..23: mol_type = other DNA
ggttagaccagatctgagcctgg

SEQ ID NO: 92 - DNA, 23 bp, synthetic construct
  misc_feature 1..23: note = Description of Artificial Sequence: Synthetic oligonucleotide
  source 1..23: mol_type = other DNA
tgctacaagggactttccgctgg

SEQ ID NO: 93 - DNA, 23 bp, synthetic construct
  misc_feature 1..23: note = Description of Artificial Sequence: Synthetic oligonucleotide
  source 1..23: mol_type = other DNA
agagagaagtattagagtggagg

SEQ ID NO: 94 - DNA, 23 bp, synthetic construct
  misc_feature 1..23: note = Description of Artificial Sequence: Synthetic oligonucleotide
  source 1..23: mol_type = other DNA
ttacaccctgtgagcctgcatgg

SEQ ID NO: 95 - DNA, 23 bp, synthetic construct
  misc_feature 1..23: note = Description of Artificial Sequence: Synthetic oligonucleotide
  source 1..23: mol_type = other DNA
aaggtagaagaagccaatgaagg

SEQ ID NO: 96 - DNA, 23 bp, synthetic construct
  misc_feature 1..23: note = Description of Artificial Sequence: Synthetic oligonucleotide
  source 1..23: mol_type = other DNA
atcagatatccactgacctttgg

SEQ ID NO: 97 - DNA, 23 bp, synthetic construct
  misc_feature 1..23: note = Description of Artificial Sequence: Synthetic oligonucleotide
  source 1..23: mol_type = other DNA
gacaagatatccttgatctgtgg

SEQ ID NO: 98 - DNA, 23 bp, synthetic construct
  misc_feature 1..23: note = Description of Artificial Sequence: Synthetic oligonucleotide
  source 1..23: mol_type = other DNA
gcccgtctgttgtgtgactctgg

SEQ ID NO: 99 - DNA, 23 bp, synthetic construct
  misc_feature 1..23: note = Description of Artificial Sequence: Synthetic oligonucleotide
  source 1..23: mol_type = other DNA
atctgagcctgggagctctctgg

SEQ ID NO: 100 - DNA, 23 bp, synthetic construct
  misc_feature 1..23: note = Description of Artificial Sequence: Synthetic oligonucleotide
  source 1..23: mol_type = other DNA
ctttccgctggggactttccagg

SEQ ID NO: 101 - DNA, 23 bp, synthetic construct
  misc_feature 1..23: note = Description of Artificial Sequence: Synthetic oligonucleotide
  source 1..23: mol_type = other DNA
cagaactacacaccagggccagg

SEQ ID NO: 102 - DNA, 23 bp, synthetic construct
  misc_feature 1..23: note = Description of Artificial Sequence: Synthetic oligonucleotide
  source 1..23: mol_type = other DNA
cctgcatgggatggatgacccgg

SEQ ID NO: 103 - DNA, 23 bp, synthetic construct
  misc_feature 1..23: note = Description of Artificial Sequence: Synthetic oligonucleotide
  source 1..23: mol_type = other DNA
ccctgtgagcctgcatgggatgg

SEQ ID NO: 104 - DNA, 23 bp, synthetic construct
  misc_feature 1..23: note = Description of Artificial Sequence: Synthetic oligonucleotide
  source 1..23: mol_type = other DNA
ctttccagggaggcgtggcctgg

SEQ ID NO: 105 - DNA, 23 bp, synthetic construct
  misc_feature 1..23: note = Description of Artificial Sequence: Synthetic oligonucleotide
  source 1..23: mol_type = other DNA
ggggactttccagggaggcgtgg

SEQ ID NO: 106 - DNA, 23 bp, synthetic construct
  misc_feature 1..23: note = Description of Artificial Sequence: Synthetic oligonucleotide
  source 1..23: mol_type = other DNA
ccgctggggactttccagggagg

SEQ ID NO: 107 - DNA, 23 bp, synthetic construct
  misc_feature 1..23: note = Description of Artificial Sequence: Synthetic oligonucleotide
  source 1..23: mol_type = other DNA
catggcccgagagctgcatccgg

SEQ ID NO: 108 - DNA, 23 bp, synthetic construct
  misc_feature 1..23: note = Description of Artificial Sequence: Synthetic oligonucleotide
  source 1..23: mol_type = other DNA
gcctgggcgggactggggagtgg

SEQ ID NO: 109 - DNA, 23 bp, synthetic construct
  misc_feature 1..23: note = Description of Artificial Sequence: Synthetic oligonucleotide
  source 1..23: mol_type = other DNA
aggcgtggcctgggcgggactgg

SEQ ID NO: 110 - DNA, 23 bp, synthetic construct
  misc_feature 1..23: note = Description of Artificial Sequence: Synthetic oligonucleotide
  source 1..23: mol_type = other DNA
gcgtggcctgggcgggactgggg

SEQ ID NO: 111 - DNA, 23 bp, synthetic construct
  misc_feature 1..23: note = Description of Artificial Sequence: Synthetic oligonucleotide
  source 1..23: mol_type = other DNA
ccagggaggcgtggcctgggcgg

SEQ ID NO: 112 - DNA, 23 bp, synthetic construct
  misc_feature 1..23: note = Description of Artificial Sequence: Synthetic oligonucleotide
  source 1..23: mol_type = other DNA
tgtggtagatccacagatcaagg

SEQ ID NO: 113 - DNA, 23 bp, synthetic construct
  misc_feature 1..23: note = Description of Artificial Sequence: Synthetic oligonucleotide
  source 1..23: mol_type = other DNA
ggtgtgtagttctgccaatcagg

SEQ ID NO: 114 - DNA, 23 bp, synthetic construct
  misc_feature 1..23: note = Description of Artificial Sequence: Synthetic oligonucleotide
  source 1..23: mol_type = other DNA
gtcagtggatatctgatccctgg

SEQ ID NO: 115 - DNA, 23 bp, synthetic construct
  misc_feature 1..23: note = Description of Artificial Sequence: Synthetic oligonucleotide
  source 1..23: mol_type = other DNA
tagcaccatccaaaggtcagtgg

SEQ ID NO: 116 - DNA, 23 bp, synthetic construct
  misc_feature 1..23: note = Description of Artificial Sequence: Synthetic oligonucleotide
  source 1..23: mol_type = other DNA
tagcttgtagcaccatccaaagg

SEQ ID NO: 117 - DNA, 23 bp, synthetic construct
  misc_feature 1..23: note = Description of Artificial Sequence: Synthetic oligonucleotide
  source 1..23: mol_type = other DNA
tctaccttctcttgctcaactgg

SEQ ID NO: 118 - DNA, 23 bp, synthetic construct
  misc_feature 1..23: note = Description of Artificial Sequence: Synthetic oligonucleotide
  source 1..23: mol_type = other DNA
cactctaatacttctctctccgg

SEQ ID NO: 119 - DNA, 23 bp, synthetic construct
  misc_feature 1..23: note = Description of Artificial Sequence: Synthetic oligonucleotide
  source 1..23: mol_type = other DNA
ccatgtgatgaaatgctaggcgg

SEQ ID NO: 120 - DNA, 23 bp, synthetic construct
  misc_feature 1..23: note = Description of Artificial Sequence: Synthetic oligonucleotide
  source 1..23: mol_type = other DNA
gggccatgtgatgaaatgctagg

SEQ ID NO: 121 - DNA, 23 bp, synthetic construct
  misc_feature 1..23: note = Description of Artificial Sequence: Synthetic oligonucleotide
  source 1..23: mol_type = other DNA
cagcagttcttgaagtactccgg

SEQ ID NO: 122 - DNA, 23 bp, synthetic construct
  misc_feature 1..23: note = Description of Artificial Sequence: Synthetic oligonucleotide
  source 1..23: mol_type = other DNA
ctgcttatatgcagcatctgagg

SEQ ID NO: 123 - DNA, 23 bp, synthetic construct
  misc_feature 1..23: note = Description of Artificial Sequence: Synthetic oligonucleotide
  source 1..23: mol_type = other DNA
cacactacttgaagcactcaagg

SEQ ID NO: 124 - DNA, 23 bp, synthetic construct
  misc_feature 1..23: note = Description of Artificial Sequence: Synthetic oligonucleotide
  source 1..23: mol_type = other DNA
taccagagtcacacaacagacgg

SEQ ID NO: 125 - DNA, 23 bp, synthetic construct
  misc_feature 1..23: note = Description of Artificial Sequence: Synthetic oligonucleotide
  source 1..23: mol_type = other DNA
acactgactaaaagggtctgagg

SEQ ID NO: 126 - DNA, 23 bp, synthetic construct
  misc_feature 1..23: note = Description of Artificial Sequence: Synthetic oligonucleotide
  source 1..23: mol_type = other DNA
caaggatatcttgtcttcgttgg

SEQ ID NO: 127 - DNA, 23 bp, synthetic construct
  misc_feature 1..23: note = Description of Artificial Sequence: Synthetic oligonucleotide
  source 1..23: mol_type = other DNA
cagggaagtagccttgtgtgtgg

SEQ ID NO: 128 - DNA, 23 bp, synthetic construct
  misc_feature 1..23: note = Description of Artificial Sequence: Synthetic oligonucleotide
  source 1..23: mol_type = other DNA
gcgggtgttctctccttcattgg

SEQ ID NO: 129 - DNA, 23 bp, synthetic construct
  misc_feature 1..23: note = Description of Artificial Sequence: Synthetic oligonucleotide
  source 1..23: mol_type = other DNA
tagttagccagagagctcccagg

SEQ ID NO: 130 - DNA, 23 bp, synthetic construct
  misc_feature 1..23: note = Description of Artificial Sequence: Synthetic oligonucleotide
  source 1..23: mol_type = other DNA
ctttattgaggcttaagcagtgg

SEQ ID NO: 131 - DNA, 23 bp, synthetic construct
  misc_feature 1..23: note = Description of Artificial Sequence: Synthetic oligonucleotide
  source 1..23: mol_type = other DNA
actcaaggcaagctttattgagg

SEQ ID NO: 132 - DNA, 23 bp, synthetic construct
  misc_feature 1..23: note = Description of Artificial Sequence: Synthetic oligonucleotide
  source 1..23: mol_type = other DNA
ggatatctgatccctggccctgg

SEQ ID NO: 133 - DNA, 23 bp, synthetic construct
  misc_feature 1..23: note = Description of Artificial Sequence: Synthetic oligonucleotide
  source 1..23: mol_type = other DNA
ggctcacagggtgtaacaagcgg

SEQ ID NO: 134 - DNA, 23 bp, synthetic construct
  misc_feature 1..23: note = Description of Artificial Sequence: Synthetic oligonucleotide
  source 1..23: mol_type = other DNA
tccatcccatgcaggctcacagg

SEQ ID NO: 135 - DNA, 23 bp, synthetic construct
  misc_feature 1..23: note = Description of Artificial Sequence: Synthetic oligonucleotide
  source 1..23: mol_type = other DNA
agtactccggatgcagctctcgg

SEQ ID NO: 136 - DNA, 23 bp, synthetic construct
  misc_feature 1..23: note = Description of Artificial Sequence: Synthetic oligonucleotide
  source 1..23: mol_type = other DNA
agagctcccaggctcagatctgg

SEQ ID NO: 137 - DNA, 23 bp, synthetic construct
  misc_feature 1..23: note = Description of Artificial Sequence: Synthetic oligonucleotide
  source 1..23: mol_type = other DNA
gattttccacactgactaaaagg

SEQ ID NO: 138 - DNA, 23 bp, synthetic construct
  misc_feature 1..23: note = Description of Artificial Sequence: Synthetic oligonucleotide
  source 1..23: mol_type = other DNA
ccgggtcatccatcccatgcagg

SEQ ID NO: 139 - DNA, 23 bp, synthetic construct
  misc_feature 1..23: note = Description of Artificial Sequence: Synthetic oligonucleotide
  source 1..23: mol_type = other DNA
cctccctggaaagtccccagcgg

SEQ ID NO: 140 - DNA, 23 bp, synthetic construct
  misc_feature 1..23: note = Description of Artificial Sequence: Synthetic oligonucleotide
  source 1..23: mol_type = other DNA
gccactccccagtcccgcccagg

SEQ ID NO: 141 - DNA, 23 bp, synthetic construct
  misc_feature 1..23: note = Description of Artificial Sequence: Synthetic oligonucleotide
  source 1..23: mol_type = other DNA
ccgcccaggccacgcctccctgg

SEQ ID NO: 142 - DNA, 23 bp, Human immunodeficiency virus 1
  source 1..23: mol_type = unassigned DNA
atcagatatccactgacctttgg

SEQ ID NO: 143 - DNA, 22 bp, Human immunodeficiency virus 1
  source 1..22: mol_type = unassigned DNA
tcagatatccactgacctttgg

SEQ ID NO: 144 - DNA, 22 bp, Human immunodeficiency virus 1
  source 1..22: mol_type = unassigned DNA
tcagatatccactgacctttgg

SEQ ID NO: 145 - DNA, 21 bp, Human immunodeficiency virus 1
  source 1..21: mol_type = unassigned DNA
cagatatccactgacctttgg

SEQ ID NO: 146 - DNA, 21 bp, Human immunodeficiency virus 1
  source 1..21: mol_type = unassigned DNA
cagatatccactgacctttgg

SEQ ID NO: 147 - DNA, 20 bp, Human immunodeficiency virus 1
  source 1..20: mol_type = unassigned DNA
agatatccactgacctttgg

SEQ ID NO: 148 - DNA, 20 bp, Human immunodeficiency virus 1
  source 1..20: mol_type = unassigned DNA
agatatccactgacctttgg

SEQ ID NO: 149 - DNA, 19 bp, Human immunodeficiency virus 1
  source 1..19: mol_type = unassigned DNA
gatatccactgacctttgg

SEQ ID NO: 150 - DNA, 19 bp, Human immunodeficiency virus 1
  source 1..19: mol_type = unassigned DNA
gatatccactgacctttgg

SEQ ID NO: 151 - DNA, 18 bp, Human immunodeficiency virus 1
  source 1..18: mol_type = unassigned DNA
atatccactgacctttgg

SEQ ID NO: 152 - DNA, 18 bp, Human immunodeficiency virus 1
  source 1..18: mol_type = unassigned DNA
atatccactgacctttgg

SEQ ID NO: 153 - DNA, 17 bp, Human immunodeficiency virus 1
  source 1..17: mol_type = unassigned DNA
tatccactgaccttggg

SEQ ID NO: 154 - DNA, 17 bp, Human immunodeficiency virus 1
  source 1..17: mol_type = unassigned DNA
tatccactgacctttgg

SEQ ID NO: 155 - DNA, 17 bp, Human immunodeficiency virus 1
  source 1..17: mol_type = unassigned DNA
tatccactgacctttgg

SEQ ID NO: 156 - DNA, 17 bp, Human immunodeficiency virus 1
  source 1..17: mol_type = unassigned DNA
tatccactgaccttaag

SEQ ID NO: 157 - DNA, 17 bp, Human immunodeficiency virus 1
  source 1..17: mol_type = unassigned DNA
tatccactgaccttgag

SEQ ID NO: 158 - DNA, 16 bp, Human immunodeficiency virus 1
  source 1..16: mol_type = unassigned DNA
atccactgaccttagg

SEQ ID NO: 159 - DNA, 16 bp, Human immunodeficiency virus 1
  source 1..16: mol_type = unassigned DNA
atccactgaccttagg

SEQ ID NO: 160 - DNA, 16 bp, Human immunodeficiency virus 1
  source 1..16: mol_type = unassigned DNA
atccactgaccttggg

SEQ ID NO: 161 - DNA, 16 bp, Human immunodeficiency virus 1
  source 1..16: mol_type = unassigned DNA
atccactgaccttggg

SEQ ID NO: 162 - DNA, 16 bp, Human immunodeficiency virus 1
  source 1..16: mol_type = unassigned DNA
atccactgaccttggg

SEQ ID NO: 163 - DNA, 16 bp, Human immunodeficiency virus 1
  source 1..16: mol_type = unassigned DNA
atccactgaccttggg

SEQ ID NO: 164 - DNA, 16 bp, Human immunodeficiency virus 1
  source 1..16: mol_type = unassigned DNA
atccactgacctttgg

SEQ ID NO: 165 - DNA, 16 bp, Human immunodeficiency virus 1
  source 1..16: mol_type = unassigned DNA
atccactgacctttgg

SEQ ID NO: 166 - DNA, 16 bp, Human immunodeficiency virus 1
  source 1..16: mol_type = unassigned DNA
atccactgacctttgg

SEQ ID NO: 167 - DNA, 16 bp, Human immunodeficiency virus 1
  source 1..16: mol_type = unassigned DNA
atccactgaccttaag

SEQ ID NO: 168 - DNA, 16 bp, Human immunodeficiency virus 1
  source 1..16: mol_type = unassigned DNA
atccactgaccttaag

SEQ ID NO: 169 - DNA, 16 bp, Human immunodeficiency virus 1
  source 1..16: mol_type = unassigned DNA
atccactgaccttcag

SEQ ID NO: 170 - DNA, 16 bp, Human immunodeficiency virus 1
  source 1..16: mol_type = unassigned DNA
atccactgaccttcag

SEQ ID NO: 171 - DNA, 16 bp, Human immunodeficiency virus 1
  source 1..16: mol_type = unassigned DNA
atccactgaccttgag

SEQ ID NO: 172 - DNA, 16 bp, Human immunodeficiency virus 1
  source 1..16: mol_type = unassigned DNA
atccactgaccttgag

SEQ ID NO: 173 - DNA, 15 bp, Human immunodeficiency virus 1
  source 1..15: mol_type = unassigned DNA
tccactgaccttagg

SEQ ID NO: 174 - DNA, 15 bp, Human immunodeficiency virus 1
  source 1..15: mol_type = unassigned DNA
tccactgaccttagg

SEQ ID NO: 175 - DNA, 15 bp, Human immunodeficiency virus 1
  source 1..15: mol_type = unassigned DNA
tccactgaccttagg

SEQ ID NO: 176 - DNA, 15 bp, Human immunodeficiency virus 1
  source 1..15: mol_type = unassigned DNA
tccactgaccttagg

SEQ ID NO: 177 - DNA, 15 bp, Human immunodeficiency virus 1
  source 1..15: mol_type = unassigned DNA
tccactgaccttagg

SEQ ID NO: 178 - DNA, 15 bp, Human immunodeficiency virus 1
  source 1..15: mol_type = unassigned DNA
tccactgaccttagg

SEQ ID NO: 179 - DNA, 15 bp, Human immunodeficiency virus 1
  source 1..15: mol_type = unassigned DNA
tccactgaccttggg

SEQ ID NO: 180 - DNA, 15 bp, Human immunodeficiency virus 1
  source 1..15: mol_type = unassigned DNA
tccactgaccttggg

SEQ ID NO: 181 - DNA, 15 bp, Human immunodeficiency virus 1
  source 1..15: mol_type = unassigned DNA
tccactgaccttggg

SEQ ID NO: 182 - DNA, 15 bp, Human immunodeficiency virus 1
  source 1..15: mol_type = unassigned DNA
tccactgaccttggg

SEQ ID NO: 183 - DNA, 15 bp, Human immunodeficiency virus 1
  source 1..15: mol_type = unassigned DNA
tccactgaccttggg

SEQ ID NO: 184 - DNA, 15 bp, Human immunodeficiency virus 1
  source 1..15: mol_type = unassigned DNA
tccactgaccttggg

SEQ ID NO: 185 - DNA, 15 bp, Human immunodeficiency virus 1
  source 1..15: mol_type = unassigned DNA
tccactgaccttggg

SEQ ID NO: 186 - DNA, 15 bp, Human immunodeficiency virus 1
  source 1..15: mol_type = unassigned DNA
tccactgaccttggg

SEQ ID NO: 187 - DNA, 15 bp, Human immunodeficiency virus 1
  source 1..15: mol_type = unassigned DNA
tccactgacctttgg

SEQ ID NO: 188 - DNA, 15 bp, Human immunodeficiency virus 1
  source 1..15: mol_type = unassigned DNA
tccactgacctttgg

SEQ ID NO: 189 - DNA, 15 bp, Human immunodeficiency virus 1
  source 1..15: mol_type = unassigned DNA
tccactgacctttgg

SEQ ID NO: 190 - DNA, 15 bp, Human immunodeficiency virus 1
  source 1..15: mol_type = unassigned DNA
tccactgacctttgg

SEQ ID NO: 191 - DNA, 15 bp, Human immunodeficiency virus 1
  source 1..15: mol_type = unassigned DNA
tccactgacctttgg

SEQ ID NO: 192 - DNA, 15 bp, Human immunodeficiency virus 1
  source 1..15: mol_type = unassigned DNA
tccactgacctttgg

SEQ ID NO: 193 - DNA, 15 bp, Human immunodeficiency virus 1
  source 1..15: mol_type = unassigned DNA
tccactgacctttgg

SEQ ID NO: 194 - DNA, 15 bp, Human immunodeficiency virus 1
  source 1..15: mol_type = unassigned DNA
tccactgacctttgg

SEQ ID NO: 195 - DNA, 15 bp, Human immunodeficiency virus 1
  source 1..15: mol_type = unassigned DNA
tccactgacctttgg

SEQ ID NO: 196 - DNA, 15 bp, Human immunodeficiency virus 1
  source 1..15: mol_type = unassigned DNA
tccactgaccttaag

SEQ ID NO: 197 - DNA, 15 bp, Human immunodeficiency virus 1
  source 1..15: mol_type = unassigned DNA
tccactgaccttaag

SEQ ID NO: 198 - DNA, 15 bp, Human immunodeficiency virus 1
  source 1..15: mol_type = unassigned DNA
tccactgaccttaag

SEQ ID NO: 199 - DNA, 15 bp, Human immunodeficiency virus 1
  source 1..15: mol_type = unassigned DNA
tccactgaccttaag

SEQ ID NO: 200 - DNA, 15 bp, Human immunodeficiency virus 1
  source 1..15: mol_type = unassigned DNA
tccactgaccttaag

SEQ ID NO: 201 - DNA, 15 bp, Human immunodeficiency virus 1
  source 1..15: mol_type = unassigned DNA
tccactgaccttcag

SEQ ID NO: 202 - DNA, 15 bp, Human immunodeficiency virus 1
  source 1..15: mol_type = unassigned DNA
tccactgaccttcag

SEQ ID NO: 203 - DNA, 15 bp, Human immunodeficiency virus 1
  source 1..15: mol_type = unassigned DNA
tccactgaccttcag

SEQ ID NO: 204 - DNA, 15 bp, Human immunodeficiency virus 1
  source 1..15: mol_type = unassigned DNA
tccactgaccttcag

SEQ ID NO: 205 - DNA, 15 bp, Human immunodeficiency virus 1
  source 1..15: mol_type = unassigned DNA
tccactgaccttcag

SEQ ID NO: 206 - DNA, 15 bp, Human immunodeficiency virus 1
  source 1..15: mol_type = unassigned DNA
tccactgaccttcag

SEQ ID NO: 207 - DNA, 15 bp, Human immunodeficiency virus 1
  source 1..15: mol_type = unassigned DNA
tccactgaccttcag

SEQ ID NO: 208 - DNA, 15 bp, Human immunodeficiency virus 1
  source 1..15: mol_type = unassigned DNA
tccactgaccttcag

SEQ ID NO: 209 - DNA, 15 bp, Human immunodeficiency virus 1
  source 1..15: mol_type = unassigned DNA
tccactgaccttcag

SEQ ID NO: 210 - DNA, 15 bp, Human immunodeficiency virus 1
  source 1..15: mol_type = unassigned DNA
tccactgaccttcag

SEQ ID NO: 211 - DNA, 15 bp, Human immunodeficiency virus 1
  source 1..15: mol_type = unassigned DNA
tccactgaccttcag

SEQ ID NO: 212 - DNA, 15 bp, Human immunodeficiency virus 1
  source 1..15: mol_type = unassigned DNA
tccactgaccttcag

SEQ ID NO: 213 - DNA, 15 bp, Human immunodeficiency virus 1
  source 1..15: mol_type = unassigned DNA
tccactgaccttgag

SEQ ID NO: 214 - DNA, 15 bp, Human immunodeficiency virus 1
  source 1..15: mol_type = unassigned DNA
tccactgaccttgag

SEQ ID NO: 215 - DNA, 15 bp, Human immunodeficiency virus 1
  source 1..15: mol_type = unassigned DNA
tccactgaccttgag

SEQ ID NO: 216 - DNA, 15 bp, Human immunodeficiency virus 1
  source 1..15: mol_type = unassigned DNA
tccactgaccttgag

SEQ ID NO: 217 - DNA, 15 bp, Human immunodeficiency virus 1
  source 1..15: mol_type = unassigned DNA
tccactgaccttgag

SEQ ID NO: 218 - DNA, 15 bp, Human immunodeficiency virus 1
  source 1..15: mol_type = unassigned DNA
tccactgaccttgag

SEQ ID NO: 219 - DNA, 15 bp, Human immunodeficiency virus 1
  source 1..15: mol_type = unassigned DNA
tccactgaccttgag

SEQ ID NO: 220 - DNA, 15 bp, Human immunodeficiency virus 1
  source 1..15: mol_type = unassigned DNA
tccactgaccttgag

SEQ ID NO: 221 - DNA, 15 bp, Human immunodeficiency virus 1
  source 1..15: mol_type = unassigned DNA
tccactgaccttgag

SEQ ID NO: 222 - DNA, 15 bp, Human immunodeficiency virus 1
  source 1..15: mol_type = unassigned DNA
tccactgacctttag

SEQ ID NO: 223 - DNA, 15 bp, Human immunodeficiency virus 1
  source 1..15: mol_type = unassigned DNA
tccactgacctttag

SEQ ID NO: 224 - DNA, 15 bp, Human immunodeficiency virus 1
  source 1..15: mol_type = unassigned DNA
tccactgacctttag

SEQ ID NO: 225 - DNA, 15 bp, Human immunodeficiency virus 1
  source 1..15: mol_type = unassigned DNA
tccactgacctttag

SEQ ID NO: 226 - DNA, 15 bp, Human immunodeficiency virus 1
  source 1..15: mol_type = unassigned DNA
tccactgacctttag

SEQ ID NO: 227 - DNA, 23 bp, Human immunodeficiency virus 1
  source 1..23: mol_type = unassigned DNA
cagcagttcttgaagtactccgg

SEQ ID NO: 228 - DNA, 22 bp, Human immunodeficiency virus 1
  source 1..22: mol_type = unassigned DNA
agcagttcttgaagtactccgg

SEQ ID NO: 229 - DNA, 21 bp, Human immunodeficiency virus 1
  source 1..21: mol_type = unassigned DNA
gcagttcttgaagtactccgg

SEQ ID NO: 230 - DNA, 20 bp, Human immunodeficiency virus 1
  source 1..20: mol_type = unassigned DNA
cagttcttgaagtactccgg

SEQ ID NO: 231 - DNA, 19 bp, Human immunodeficiency virus 1
  source 1..19: mol_type = unassigned DNA
agttcttgaagtactccgg

SEQ ID NO: 232 - DNA, 18 bp, Human immunodeficiency virus 1
  source 1..18: mol_type = unassigned DNA
gttcttgaagtactccgg

SEQ ID NO: 233 - DNA, 17 bp, Human immunodeficiency virus 1
  source 1..17: mol_type = unassigned DNA
ttcttgaagtactccgg

SEQ ID NO: 234 - DNA, 16 bp, Human immunodeficiency virus 1
  source 1..16: mol_type = unassigned DNA
tcttgaagtactccgg

SEQ ID NO: 235 - DNA, 16 bp, Human immunodeficiency virus 1
  source 1..16: mol_type = unassigned DNA
tcttgaagtactctag

SEQ ID NO: 236 - DNA, 15 bp, Human immunodeficiency virus 1
  source 1..15: mol_type = unassigned DNA
cttgaagtactcagg

SEQ ID NO: 237 - DNA, 15 bp, Human immunodeficiency virus 1
  source 1..15: mol_type = unassigned DNA
cttgaagtactcagg

SEQ ID NO: 238 - DNA, 15 bp, Human immunodeficiency virus 1
  source 1..15: mol_type = unassigned DNA
cttgaagtactcagg

SEQ ID NO: 239 - DNA, 15 bp, Human immunodeficiency virus 1
  source 1..15: mol_type = unassigned DNA
cttgaagtactcagg

SEQ ID NO: 240 - DNA, 15 bp, Human immunodeficiency virus 1
  source 1..15: mol_type = unassigned DNA
cttgaagtactccgg

SEQ ID NO: 241 - DNA, 15 bp, Human immunodeficiency virus 1
  source 1..15: mol_type = unassigned DNA
cttgaagtactctgg

SEQ ID NO: 242 - DNA, 15 bp, Human immunodeficiency virus 1
  source 1..15: mol_type = unassigned DNA
cttgaagtactcaag

SEQ ID NO: 243 - DNA, 15 bp, Human immunodeficiency virus 1
  source 1..15: mol_type = unassigned DNA
cttgaagtactcaag

SEQ ID NO: 244 - DNA, 15 bp, Human immunodeficiency virus 1
  source 1..15: mol_type = unassigned DNA
cttgaagtactcaag

SEQ ID NO: 245 - DNA, 15 bp, Human immunodeficiency virus 1
  source 1..15: mol_type = unassigned DNA
cttgaagtactcaag

SEQ ID NO: 246 - DNA, 15 bp, Human immunodeficiency virus 1
  source 1..15: mol_type = unassigned DNA
cttgaagtactcaag

SEQ ID NO: 247 - DNA, 15 bp, Human immunodeficiency virus 1
  source 1..15: mol_type = unassigned DNA
cttgaagtactccag

SEQ ID NO: 248 - DNA, 15 bp, Human immunodeficiency virus 1
  source 1..15: mol_type = unassigned DNA
cttgaagtactccag

SEQ ID NO: 249 - DNA, 15 bp, Human immunodeficiency virus 1
  source 1..15: mol_type = unassigned DNA
cttgaagtactccag

SEQ ID NO: 250 - DNA, 15 bp, Human immunodeficiency virus 1
  source 1..15: mol_type = unassigned DNA
cttgaagtactccag

SEQ ID NO: 251 - DNA, 15 bp, Human immunodeficiency virus 1
  source 1..15: mol_type = unassigned DNA
cttgaagtactctag

SEQ ID NO: 252 - DNA, 15 bp, Human immunodeficiency virus 1
  source 1..15: mol_type = unassigned DNA
cttgaagtactctag

SEQ ID NO: 253 - DNA, 23 bp, Human immunodeficiency virus 1
  source 1..23: mol_type = unassigned DNA
atcagatatccactgacctttgg

SEQ ID NO: 254 - DNA, 22 bp, Human immunodeficiency virus 1
  source 1..22: mol_type = unassigned DNA
tcagatatccactgacctttgg

SEQ ID NO: 255 - DNA, 22 bp, Human immunodeficiency virus 1
  source 1..22: mol_type = unassigned DNA
tcagatatccactgacctttgg

SEQ ID NO: 256 - DNA, 21 bp, Human immunodeficiency virus 1
  source 1..21: mol_type = unassigned DNA
cagatatccactgacctttgg

SEQ ID NO: 257 - DNA, 21 bp, Human immunodeficiency virus 1
  source 1..21: mol_type = unassigned DNA
cagatatccactgacctttgg

SEQ ID NO: 258 - DNA, 20 bp, Human immunodeficiency virus 1
  source 1..20: mol_type = unassigned DNA
agatatccactgacctttgg

SEQ ID NO: 259 - DNA, 20 bp, Human immunodeficiency virus 1
  source 1..20: mol_type = unassigned DNA
agatatccactgacctttgg

SEQ ID NO: 260 - DNA, 19 bp, Human immunodeficiency virus 1
  source 1..19: mol_type = unassigned DNA
gatatccactgacctttgg

SEQ ID NO: 261 - DNA, 19 bp, Human immunodeficiency virus 1
  source 1..19: mol_type = unassigned DNA
gatatccactgacctttgg

SEQ ID NO: 262 - DNA, 18 bp, Human immunodeficiency virus 1
  source 1..18: mol_type = unassigned DNA
atatccactgacctttgg

SEQ ID NO: 263 - DNA, 18 bp, Human immunodeficiency virus 1
  source 1..18: mol_type = unassigned DNA
atatccactgacctttgg

SEQ ID NO: 264 - DNA, 17 bp, Human immunodeficiency virus 1
  source 1..17: mol_type = unassigned DNA
tatccactgaccttggg

SEQ ID NO: 265 - DNA, 17 bp, Human immunodeficiency virus 1
  source 1..17: mol_type = unassigned DNA
tatccactgacctttgg

SEQ ID NO: 266 - DNA, 17 bp, Human immunodeficiency virus 1
  source 1..17: mol_type = unassigned DNA
tatccactgacctttgg

SEQ ID NO: 267 - DNA, 17 bp, Human immunodeficiency virus 1
  source 1..17: mol_type = unassigned DNA
tatccactgaccttaag

SEQ ID NO: 268 - DNA, 17 bp, Human immunodeficiency virus 1
  source 1..17: mol_type = unassigned DNA
tatccactgaccttgag

SEQ ID NO: 269 - DNA, 16 bp, Human immunodeficiency virus 1
  source 1..16: mol_type = unassigned DNA
atccactgaccttagg

SEQ ID NO: 270 - DNA, 16 bp, Human immunodeficiency virus 1
  source 1..16: mol_type = unassigned DNA
atccactgaccttagg

SEQ ID NO: 271 - DNA, 16 bp, Human immunodeficiency virus 1
  source 1..16: mol_type = unassigned DNA
atccactgaccttggg

SEQ ID NO: 272 - DNA, 16 bp, Human immunodeficiency virus 1
  source 1..16: mol_type = unassigned DNA
atccactgaccttggg

SEQ ID NO: 273 - DNA, 16 bp, Human immunodeficiency virus 1
  source 1..16: mol_type = unassigned DNA
atccactgaccttggg

SEQ ID NO: 274 - DNA, 16 bp, Human immunodeficiency virus 1
  source 1..16: mol_type = unassigned DNA
atccactgaccttggg

SEQ ID NO: 275 - DNA, 16 bp, Human immunodeficiency virus 1
  source 1..16: mol_type = unassigned DNA
atccactgacctttgg

SEQ ID NO: 276 - DNA, 16 bp, Human immunodeficiency virus 1
  source 1..16: mol_type = unassigned DNA
atccactgacctttgg

SEQ ID NO: 277 - DNA, 16 bp, Human immunodeficiency virus 1
  source 1..16: mol_type = unassigned DNA
atccactgacctttgg

SEQ ID NO: 278 - DNA, 16 bp, Human immunodeficiency virus 1
  source 1..16: mol_type = unassigned DNA
atccactgaccttaag

SEQ ID NO: 279 - DNA, 16 bp, Human immunodeficiency virus 1
  source 1..16: mol_type = unassigned DNA
atccactgaccttaag

SEQ ID NO: 280 - DNA, 16 bp, Human immunodeficiency virus 1
  source 1..16: mol_type = unassigned DNA
atccactgaccttcag

SEQ ID NO: 281 - DNA, 16 bp, Human immunodeficiency virus 1
  source 1..16: mol_type = unassigned DNA
atccactgaccttcag

SEQ ID NO: 282 - DNA, 16 bp, Human immunodeficiency virus 1
  source 1..16: mol_type = unassigned DNA
atccactgaccttgag

SEQ ID NO: 283 - DNA, 16 bp, Human immunodeficiency virus 1
  source 1..16: mol_type = unassigned DNA
atccactgaccttgag

SEQ ID NO: 284 - DNA, 15 bp, Human immunodeficiency virus 1
  source 1..15: mol_type = unassigned DNA
tccactgaccttagg

SEQ ID NO: 285 - DNA, 15 bp, Human immunodeficiency virus 1
  source 1..15: mol_type = unassigned DNA
tccactgaccttagg

SEQ ID NO: 286 - DNA, 15 bp, Human immunodeficiency virus 1
  source 1..15: mol_type = unassigned DNA
tccactgaccttagg

SEQ ID NO: 287 - DNA, 15 bp, Human immunodeficiency virus 1
  source 1..15: mol_type = unassigned DNA
tccactgaccttagg

SEQ ID NO: 288 - DNA, 15 bp, Human immunodeficiency virus 1
  source 1..15: mol_type = unassigned DNA
tccactgaccttagg

SEQ ID NO: 289 - DNA, 15 bp, Human immunodeficiency virus 1
  source 1..15: mol_type = unassigned DNA
tccactgaccttagg

SEQ ID NO: 290 - DNA, 15 bp, Human immunodeficiency virus 1
  source 1..15: mol_type = unassigned DNA
tccactgaccttggg

SEQ ID NO: 291 - DNA, 15 bp, Human immunodeficiency virus 1
  source 1..15: mol_type = unassigned DNA
tccactgaccttggg

SEQ ID NO: 292 - DNA, 15 bp, Human immunodeficiency virus 1
  source 1..15: mol_type = unassigned DNA
tccactgaccttggg

SEQ ID NO: 293 - DNA, 15 bp, Human immunodeficiency virus 1
  source 1..15: mol_type = unassigned DNA
tccactgaccttggg

SEQ ID NO: 294 - DNA, 15 bp, Human immunodeficiency virus 1
  source 1..15: mol_type = unassigned DNA
tccactgaccttggg

SEQ ID NO: 295 - DNA, 15 bp, Human immunodeficiency virus 1
  source 1..15: mol_type = unassigned DNA
tccactgaccttggg

SEQ ID NO: 296 - DNA, 15 bp, Human immunodeficiency virus 1
  source 1..15: mol_type = unassigned DNA
tccactgaccttggg

SEQ ID NO: 297 - DNA, 15 bp, Human immunodeficiency virus 1
  source 1..15: mol_type = unassigned DNA
tccactgaccttggg

SEQ ID NO: 298 - DNA, 15 bp, Human immunodeficiency virus 1
  source 1..15: mol_type = unassigned DNA
tccactgacctttgg

SEQ ID NO: 299 - DNA, 15 bp, Human immunodeficiency virus 1
  source 1..15: mol_type = unassigned DNA
tccactgacctttgg

SEQ ID NO: 300 - DNA, 15 bp, Human immunodeficiency virus 1
  source 1..15: mol_type = unassigned DNA
tccactgacctttgg

SEQ ID NO: 301 - DNA, 15 bp, Human immunodeficiency virus 1
  source 1..15: mol_type = unassigned DNA
tccactgacctttgg

SEQ ID NO: 302 - DNA, 15 bp, Human immunodeficiency virus 1
  source 1..15: mol_type = unassigned DNA
tccactgacctttgg

SEQ ID NO: 303 - DNA, 15 bp, Human immunodeficiency virus 1
  source 1..15: mol_type = unassigned DNA
tccactgacctttgg

SEQ ID NO: 304 - DNA, 15 bp, Human immunodeficiency virus 1
  source 1..15: mol_type = unassigned DNA
tccactgacctttgg

SEQ ID NO: 305 - DNA, 15 bp, Human immunodeficiency virus 1
  source 1..15: mol_type = unassigned DNA
tccactgacctttgg

SEQ ID NO: 306 - DNA, 15 bp, Human immunodeficiency virus 1
  source 1..15: mol_type = unassigned DNA
tccactgacctttgg

SEQ ID NO: 307 - DNA, 15 bp, Human immunodeficiency virus 1
  source 1..15: mol_type = unassigned DNA
tccactgaccttaag

SEQ ID NO: 308 - DNA, 15 bp, Human immunodeficiency virus 1
  source 1..15: mol_type = unassigned DNA
tccactgaccttaag

SEQ ID NO: 309 - DNA, 15 bp, Human immunodeficiency virus 1
  source 1..15: mol_type = unassigned DNA
tccactgaccttaag

SEQ ID NO: 310 - DNA, 15 bp, Human immunodeficiency virus 1
  source 1..15: mol_type = unassigned DNA
tccactgaccttaag

SEQ ID NO: 311 - DNA, 15 bp, Human immunodeficiency virus 1
  source 1..15: mol_type = unassigned DNA
tccactgaccttaag

SEQ ID NO: 312 - DNA, 15 bp, Human immunodeficiency virus 1
  source 1..15: mol_type = unassigned DNA
tccactgaccttcag

SEQ ID NO: 313 - DNA, 15 bp, Human immunodeficiency virus 1
  source 1..15: mol_type = unassigned DNA
tccactgaccttcag

SEQ ID NO: 314 - DNA, 15 bp, Human immunodeficiency virus 1
  source 1..15: mol_type = unassigned DNA
tccactgaccttcag

SEQ ID NO: 315 - DNA, 15 bp, Human immunodeficiency virus 1
  source 1..15: mol_type = unassigned DNA
tccactgaccttcag

SEQ ID NO: 316 - DNA, 15 bp, Human immunodeficiency virus 1
  source 1..15: mol_type = unassigned DNA
tccactgaccttcag

SEQ ID NO: 317 - DNA, 15 bp, Human immunodeficiency virus 1
  source 1..15: mol_type = unassigned DNA
tccactgaccttcag

SEQ ID NO: 318 - DNA, 15 bp, Human immunodeficiency virus 1
  source 1..15: mol_type = unassigned DNA
tccactgaccttcag

SEQ ID NO: 319 - DNA, 15 bp, Human immunodeficiency virus 1
  source 1..15: mol_type = unassigned DNA
tccactgaccttcag

SEQ ID NO: 320 - DNA, 15 bp, Human immunodeficiency virus 1
  source 1..15: mol_type = unassigned DNA
tccactgaccttcag

SEQ ID NO: 321 - DNA, 15 bp, Human immunodeficiency virus 1
  source 1..15: mol_type = unassigned DNA
tccactgaccttcag

SEQ ID NO: 322 - DNA, 15 bp, Human immunodeficiency virus 1
  source 1..15: mol_type = unassigned DNA
tccactgaccttcag

SEQ ID NO: 323 - DNA, 15 bp, Human immunodeficiency virus 1
  source 1..15: mol_type = unassigned DNA
tccactgaccttcag

SEQ ID NO: 324 - DNA, 15 bp, Human immunodeficiency virus 1
  source 1..15: mol_type = unassigned DNA
tccactgaccttgag

SEQ ID NO: 325 - DNA, 15 bp, Human immunodeficiency virus 1
  source 1..15: mol_type = unassigned DNA
tccactgaccttgag

SEQ ID NO: 326 - DNA, 15 bp, Human immunodeficiency virus 1
  source 1..15: mol_type = unassigned DNA
tccactgaccttgag

SEQ ID NO: 327 - DNA, 15 bp, Human immunodeficiency virus 1
  source 1..15: mol_type = unassigned DNA
tccactgaccttgag

SEQ ID NO: 328 - DNA, 15 bp, Human immunodeficiency virus 1
  source 1..15: mol_type = unassigned DNA
tccactgaccttgag

SEQ ID NO: 329 - DNA, 15 bp, Human immunodeficiency virus 1
  source 1..15: mol_type = unassigned DNA
tccactgaccttgag

SEQ ID NO: 330 - DNA, 15 bp, Human immunodeficiency virus 1
  source 1..15: mol_type = unassigned DNA
tccactgaccttgag

SEQ ID NO: 331 - DNA, 15 bp, Human immunodeficiency virus 1
  source 1..15: mol_type = unassigned DNA
tccactgaccttgag

SEQ ID NO: 332 - DNA, 15 bp, Human immunodeficiency virus 1
  source 1..15: mol_type = unassigned DNA
tccactgaccttgag

SEQ ID NO: 333 - DNA, 15 bp, Human immunodeficiency virus 1
  source 1..15: mol_type = unassigned DNA
tccactgacctttag

SEQ ID NO: 334 - DNA, 15 bp, Human immunodeficiency virus 1
  source 1..15: mol_type = unassigned DNA
tccactgacctttag

SEQ ID NO: 335 - DNA, 15 bp, Human immunodeficiency virus 1
  source 1..15: mol_type = unassigned DNA
tccactgacctttag

SEQ ID NO: 336 - DNA, 15 bp, Human immunodeficiency virus 1
  source 1..15: mol_type = unassigned DNA
tccactgacctttag

SEQ ID NO: 337 - DNA, 15 bp, Human immunodeficiency virus 1
  source 1..15: mol_type = unassigned DNA
tccactgacctttag

SEQ ID NO: 338 - DNA, 23 bp, Human immunodeficiency virus 1
  source 1..23: mol_type = unassigned DNA
cagcagttcttgaagtactccgg

SEQ ID NO: 339 - DNA, 22 bp, Human immunodeficiency virus 1
  source 1..22: mol_type = unassigned DNA
agcagttcttgaagtactccgg

SEQ ID NO: 340 - DNA, 21 bp, Human immunodeficiency virus 1
  source 1..21: mol_type = unassigned DNA
gcagttcttgaagtactccgg

SEQ ID NO: 341 - DNA, 20 bp, Human immunodeficiency virus 1
  source 1..20: mol_type = unassigned DNA
cagttcttgaagtactccgg

SEQ ID NO: 342 - DNA, 19 bp, Human immunodeficiency virus 1
  source 1..19: mol_type = unassigned DNA
agttcttgaagtactccgg

SEQ ID NO: 343 - DNA, 18 bp, Human immunodeficiency virus 1
  source 1..18: mol_type = unassigned DNA
gttcttgaagtactccgg

SEQ ID NO: 344 - DNA, 17 bp, Human immunodeficiency virus 1
  source 1..17: mol_type = unassigned DNA
ttcttgaagtactccgg

SEQ ID NO: 345 - DNA, 16 bp, Human immunodeficiency virus 1
  source 1..16: mol_type = unassigned DNA
tcttgaagtactccgg

SEQ ID NO: 346 - DNA, 16 bp, Human immunodeficiency virus 1
  source 1..16: mol_type = unassigned DNA
tcttgaagtactctag

SEQ ID NO: 347 - DNA, 15 bp, Human immunodeficiency virus 1
  source 1..15: mol_type = unassigned DNA
cttgaagtactcagg

SEQ ID NO: 348 - DNA, 15 bp, Human immunodeficiency virus 1
  source 1..15: mol_type = unassigned DNA
cttgaagtactcagg

SEQ ID NO: 349 - DNA, 15 bp, Human immunodeficiency virus 1
  source 1..15: mol_type = unassigned DNA
cttgaagtactcagg

SEQ ID NO: 350 - DNA, 15 bp, Human immunodeficiency virus 1
  source 1..15: mol_type = unassigned DNA
cttgaagtactcagg

SEQ ID NO: 351 - DNA, 15 bp, Human immunodeficiency virus 1
  source 1..15: mol_type = unassigned DNA
cttgaagtactccgg

SEQ ID NO: 352 - DNA, 15 bp, Human immunodeficiency virus 1
  source 1..15: mol_type = unassigned DNA
cttgaagtactctgg

SEQ ID NO: 353 - DNA, 15 bp, Human immunodeficiency virus 1
  source 1..15: mol_type = unassigned DNA
cttgaagtactcaag

SEQ ID NO: 354 - DNA, 15 bp, Human immunodeficiency virus 1
  source 1..15: mol_type = unassigned DNA
cttgaagtactcaag

SEQ ID NO: 355 - DNA, 15 bp, Human immunodeficiency virus 1
  source 1..15: mol_type = unassigned DNA
cttgaagtactcaag

SEQ ID NO: 356 - DNA, 15 bp, Human immunodeficiency virus 1
  source 1..15: mol_type = unassigned DNA
cttgaagtactcaag

SEQ ID NO: 357 - DNA, 15 bp, Human immunodeficiency virus 1
  source 1..15: mol_type = unassigned DNA
cttgaagtactcaag

SEQ ID NO: 358 - DNA, 15 bp, Human immunodeficiency virus 1
  source 1..15: mol_type = unassigned DNA
cttgaagtactccag

SEQ ID NO: 359 - DNA, 15 bp, Human immunodeficiency virus 1
  source 1..15: mol_type = unassigned DNA
cttgaagtactccag

SEQ ID NO: 360 - DNA, 15 bp, Human immunodeficiency virus 1
  source 1..15: mol_type = unassigned DNA
cttgaagtactccag

SEQ ID NO: 361 - DNA, 15 bp, Human immunodeficiency virus 1
  source 1..15: mol_type = unassigned DNA
cttgaagtactccag

SEQ ID NO: 362 - DNA, 15 bp, Human immunodeficiency virus 1
  source 1..15: mol_type = unassigned DNA
cttgaagtactctag

SEQ ID NO: 363 - DNA, 15 bp, Human immunodeficiency virus 1
  source 1..15: mol_type = unassigned DNA
cttgaagtactctag

SEQ ID NO: 364 - DNA, 23 bp, Human immunodeficiency virus 1
  source 1..23: mol_type = unassigned DNA
gatctgtggatctaccacacaca

SEQ ID NO: 365 - DNA, 26 bp, Human immunodeficiency virus 1
  source 1..26: mol_type = unassigned DNA
gatctgtggatctaccacacacaagg

SEQ ID NO: 366 - DNA, 20 bp, Human immunodeficiency virus 1
  source 1..20: mol_type = unassigned DNA
gattggcagaactacacacc

SEQ ID NO: 367 - DNA, 23 bp, Human immunodeficiency virus 1
  source 1..23: mol_type = unassigned DNA
gattggcagaactacacaccagg

SEQ ID NO: 368 - DNA, 27 bp, Human immunodeficiency virus 1
  source 1..27: mol_type = unassigned DNA
gccagggatcagatatccactgacctt

SEQ ID NO: 369 - DNA, 30 bp, Human immunodeficiency virus 1; identical to SEQ ID NO: 1
  source 1..30: mol_type = unassigned DNA

SEQ ID NO: 370 - DNA, 30 bp, Human immunodeficiency virus 1
  source 1..30: mol_type = unassigned DNA
gagtacttcaagaactgctgacatcgagct

SEQ ID NO: 371 - DNA, 33 bp, Human immunodeficiency virus 1
  source 1..33: mol_type = unassigned DNA
ccggagtacttcaagaactgctgacatcgagct

SEQ ID NO: 372 - DNA, 20 bp, Human immunodeficiency virus 1
  source 1..20: mol_type = unassigned DNA
gcgtggcctgggcgggactg

SEQ ID NO: 373 - DNA, 23 bp, Human immunodeficiency virus 1
  source 1..23: mol_type = unassigned DNA
gcgtggcctgggcgggactgggg

SEQ ID NO: 374 - DNA, 22 bp, Human immunodeficiency virus 1
  source 1..22: mol_type = unassigned DNA
tcagatgctgcatataagcagc

SEQ ID NO: 375 - DNA, 25 bp, Human immunodeficiency virus 1
  source 1..25: mol_type = unassigned DNA
ccctcagatgctgcatataagcagc

SEQ ID NO: 376 - DNA, 634 bp, synthetic construct
  misc_feature 1..634: note = Description of Artificial Sequence: Synthetic polynucleotide
  source 1..634: mol_type = other DNA
tggaagggctaattcactcccaacgaagacaagatatccttgatctgtggatctaccacacacaaggctacttccctgattggcagaactacacaccagggccagggatcagatatccactgacctttggatggtgctacaagctagtaccagttgagcaagagaaggtagaagaagccaatgaaggagagaacacccgcttgttacaccctgtgagcctgcatgggatggatgacccggagagagaagtattagagtggaggtttgacagccgcctagcatttcatcacatggcccgagagctgcatccggagtacttcaagaactgctgacatcgagcttgctacaagggactttccgctggggactttccagggaggcgtggcctgggcgggactggggagtggcgagccctcagatgctgcatataagcagctgctttttgcttgtactgggtctctctggttagaccagatctgagcctgggagctctctggctaactagggaacccactgcttaagcctcaataaagcttgccttgagtgcttcaagtagtgtgtgcccgtctgttgtgtgactctggtaactagagatccctcagacccttttagtcagtgtggaaaatctctagca

SEQ ID NO: 377 - DNA, 453 bp, synthetic construct
  misc_feature 1..453: note = Description of Artificial Sequence: Synthetic polynucleotide
  source 1..453: mol_type = other DNA
tggaagggctaattcactcccaacgaagacaagatatccttgatctgtggatctaccacacacaaggctacttccctgattggcagaactacacaccagggccagggatcagatatccactgacctttggatggtgctacaagctagtaccagttgagcaagagaaggtagaagaagccaatgaaggagagaacacccgcttgttacaccctgtgagcctgcatgggatggatgacccggagagagaagtattagagtggaggtttgacagccgcctagcatttcatcacatggcccgagagctgcatccggagtacttcaagaactgctgacatcgagcttgctacaagggactttccgctggggactttccagggaggcgtggcctgggcgggactggggagtggcgagccctcagatgctgcatataagcagctgctttttgcttgtact

SEQ ID NO: 378 - DNA, 97 bp, synthetic construct
  misc_feature 1..97: note = Description of Artificial Sequence: Synthetic oligonucleotide
  source 1..97: mol_type = other DNA
gggtctctctggttagaccagatctgagcctgggagctctctggctaactagggaacccactgcttaagcctcaataaagcttgccttgagtgcttc

SEQ ID NO: 379 - DNA, 84 bp, synthetic construct
  misc_feature 1..84: note = Description of Artificial Sequence: Synthetic oligonucleotide
  source 1..84: mol_type = other DNA
aagtagtgtgtgcccgtctgttgtgtgactctggtaactagagatccctcagacccttttagtcagtgtggaaaatctctagca

SEQ ID NO: 380 - DNA, 818 bp, synthetic construct
  misc_feature 1..818: note = Description of Artificial Sequence: Synthetic polynucleotide
  source 1..818: mol_type = other DNA
tggaagggatttattacagtgcaagaagacatagaatcttagacatatacttagaaaaggaagaaggcatcataccagattggcaggattacacctcaggaccaggaattagatacccaaagacatttggctggctatggaaattagtccctgtaaatgtatcagatgaggcacaggaggatgaggagcattatttaatgcatccagctcaaacttcccagtgggatgacccttggggagaggttctagcatggaagtttgatccaactctggcctacacttatgaggcatatgttagatacccagaagagtttggaagcaagtcaggcctgtcagaggaagaggttagaagaaggctaaccgcaagaggccttcttaacatggctgacaagaaggaaactcgctgaaacagcagggactttccacaaggggatgttacggggaggtactggggaggagccggtcgggaacgcccactttcttgatgtataaatatcactgcatttcgctctgtattcagtcgctctgcggagaggctggcagattgagccctgggaggttctctccagcactagcaggtagagcctgggtgttccctgctagactctcaccagcacttggccggtgctgggcagagtgactccacgcttgcttgcttaaagccctcttcaataaagctgccattttagaagtaagctagtgtgtgttcccatctctcctagccgccgcctggtcaactcggtactcaataataagaagaccctggtctgttaggaccctttctgctttgggaaaccgaagcaggaaaatccctagca

SEQ ID NO: 381 - DNA, 517 bp, synthetic construct
  misc_feature 1..517: note = Description of Artificial Sequence: Synthetic polynucleotide
  source 1..517: mol_type = other DNA
tggaagggatttattacagtgcaagaagacatagaatcttagacatatacttagaaaaggaagaaggcatcataccagattggcaggattacacctcaggaccaggaattagatacccaaagacatttggctggctatggaaattagtccctgtaaatgtatcagatgaggcacaggaggatgaggagcattatttaatgcatccagctcaaacttcccagtgggatgacccttggggagaggttctagcatggaagtttgatccaactctggcctacacttatgaggcatatgttagatacccagaagagtttggaagcaagtcaggcctgtcagaggaagaggttagaagaaggctaaccgcaagaggccttcttaacatggctgacaagaaggaaactcgctgaaacagcagggactttccacaaggggatgttacggggaggtactggggaggagccggtcgggaacgcccactttcttgatgtataaatatcactgcatttcgctctgtatt

SEQ ID NO: 382 - DNA, 176 bp, synthetic construct
  misc_feature 1..176: note = Description of Artificial Sequence: Synthetic polynucleotide
  source 1..176: mol_type = other DNA
cagtcgctctgcggagaggctggcagattgagccctgggaggttctctccagcactagcaggtagagcctgggtgttccctgctagactctcaccagcacttggccggtgctgggcagagtgactccacgcttgcttgcttaaagccctcttcaataaagctgccattttagaagt

SEQ ID NO: 383 - DNA, 125 bp, synthetic construct
  misc_feature 1..125: note = Description of Artificial Sequence: Synthetic polynucleotide
  source 1..125: mol_type = other DNA
aagctagtgtgtgttcccatctctcctagccgccgcctggtcaactcggtactcaataataagaagaccctggtctgttaggaccctttctgctttgggaaaccgaagcaggaaaatccctagca

SEQ ID NO: 384 - DNA, 14825 bp, Human immunodeficiency virus 1
  source 1..14825: mol_type = unassigned DNA
tggaagggctaatttggtcccaaaaaagacaagagatccttgatctgtggatctaccacacacaaggctacttccctgattggcagaactacacaccagggccagggatcagatatccactgacctttggatggtgcttcaagttagtaccagttgaaccagagcaagtagaagaggccaatgaaggagagaacaacagcttgttacaccctatgagccagcatgggatggaggacccggagggagaagtattagtgtggaagtttgacagcctcctagcatttcgtcacatggcccgagagctgcatccggagtactacaaagactgctgacatcgagctttctacaagggactttccgctggggactttccagggaggtgtggcctgggcgggactggggagtggcgagccctcagatgctacatataagcagctgctttttgcctgtactgggtctctctggttagaccagatctgagcctgggagctctctggctaactagggaacccactgcttaagcctcaataaagcttgccttgagtgctcaaagtagtgtgtgcccgtctgttgtgtgactctggtaactagagatccctcagacccttttagtcagtgtggaaaatctctagcagtggcgcccgaacagggacttgaaagcgaaagtaaagccagaggagatctctcgacgcaggactcggcttgctgaagcgcgcacggcaagaggcgaggggcggcgactggtgagtacgccaaaaattttgactagcggaggctagaaggagagagatgggtgcgagagcgtcggtattaagcgggggagaattagataaatgggaaaaaattcggttaaggccagggggaaagaaacaatataaactaaaacatatagtatgggcaagcagggagctagaacgattcgcagttaatcctggccttttagagacatcagaaggctgtagacaaatactgggacagctacaaccatcccttcagacaggatcagaagaacttagatcattatataatacaatagcagtcctctattgtgtgcatcaaaggatagatgtaaaagacaccaaggaagccttagataagatagaggaagagcaaaacaaaagtaagaaaaaggcacagcaagcagcagctgacacaggaaacaacagccaggtcagccaaaattaccctatagtgcagaacctccaggggcaaatggtacatcaggccatatcacctagaactttaaatgcatgggtaaaagtagtagaagagaaggctttcagcccagaagtaatacccatgttttcagcattatcagaaggagccaccccacaagatttaaataccatgctaaacacagtggggggacatcaagcagccatgcaaatgttaaaagagaccatcaatgaggaagctgcagaatgggatagattgcatccagtgcatgcagggcctattgcaccaggccagatgagagaaccaaggggaagtgacatagcaggaactactagtacccttcaggaacaaataggatggatgacacataatccacctatcccagtaggagaaatctataaaagatggataatcctgggattaaataaaatagtaagaatgtatagccctaccagcattctggacataagacaaggaccaaaggaaccctttagagactatgtagaccgattctataaaactctaagagccgagcaagcttcacaagaggtaaaaaattggatgacagaaaccttgttggtccaaaatgcgaacccagattgtaagactattttaaaagcattgggaccaggagcgacactagaagaaatgatgacagcatgtcagggagtggggggacccggccataaagcaagagttttggctgaagcaatgagccaagtaacaaatccagctaccataatgatacagaaaggcaattttaggaaccaaagaaagactgttaagtgtttcaattgtggcaaagaagggcacatagccaaaaattgcagggcccctaggaaaaagggctgttggaaatgtggaaaggaaggacaccaaatgaaagattgtactgagagacaggctaattttttagggaagatctggccttcccacaagggaaggccagggaattttcttcagagcagaccagagccaacagccccaccagaagagagcttcaggtttggggaagagacaacaactccctctcagaagcaggagccgatagacaaggaactgtatcctttagcttccctcagatcactctttggcagcgacccctcgtcacaataaagataggggggcaattaaaggaagctctattagatacaggagcagatgatacagtattagaagaaatgaatttgccaggaagatggaaaccaaaaatgatagggggaattggaggttttatcaaagtaagacagtatgatcagatactcatagaaatctgcggacataaagctataggtacagtattagtaggacctacacctgtcaacataattggaagaaatctgttgactcagattggctgcactttaaattttcccattagtcctattgagactgtaccagtaaaattaaagccaggaatggatggcccaaaagttaaacaatggccattgacagaagaaaaaataaaagcattagtagaaatttgtacagaaatggaaaaggaaggaaaaatttcaaaaattgggcctgaaaatccatacaatactccagtatttgccataaagaaaaaagacagtactaaatggagaaaattagtagatttcagagaacttaataagagaactcaagatttctgggaagttcaattaggaataccacatcctgcagggttaaaacagaaaaaatcagtaacagtactggatgtgggcgatgcatatttttcagttcccttagataaagacttcaggaagtatactgcatttaccatacctagtataaacaatgagacaccagggattagatatcagtacaatgtgcttccacagggatggaaaggatcaccagcaatattccagtgtagcatgacaaaaatcttagagccttttagaaaacaaaatccagacatagtcatctatcaatacatggatgatttgtatgtaggatctgacttagaaatagggcagcatagaacaaaaatagaggaactgagacaacatctgttgaggtggggatttaccacaccagacaaaaaacatcagaaagaacctccattcctttggatgggttatgaactccatcctgataaatggacagtacagcctatagtgctgccagaaaaggacagctggactgtcaatgacatacagaaattagtgggaaaattgaattgggcaagtcagatttatgcagggattaaagtaaggcaattatgtaaacttcttaggggaaccaaagcactaacagaagtagtaccactaacagaagaagcagagctagaactggcagaaaacagggagattctaaaagaaccggtacatggagtgtattatgacccatcaaaagacttaatagcagaaatacagaagcaggggcaaggccaatggacatatcaaatttatcaagagccatttaaaaatctgaaaacaggaaagtatgcaagaatgaagggtgcccacactaatgatgtgaaacaattaacagaggcagtacaaaaaatagccacagaaagcatagtaatatggggaaagactcctaaatttaaattacccatacaaaaggaaacatgggaagcatggtggacagagtattggcaagccacctggattcctgagtgggagtttgtcaatacccctcccttagtgaagttatggtaccagttagagaaagaacccataataggagcagaaactttctatgtagatggggcagccaatagggaaactaaattaggaaaagcaggatatgtaactgacagaggaagacaaaaagttgtccccctaacggacacaacaaatcagaagactgagttacaagcaattcatctagctttgcaggattcgggattagaagtaaacatagtgacagactcacaatatgcattgggaatcattcaagcacaaccagataagagtgaatcagagttagtcagtcaaataatagagcagttaataaaaaaggaaaaagtctacctggcatgggtaccagcacacaaaggaattggaggaaatgaacaagtagataaattggtcagtgctggaatcaggaaagtactatttttagatggaatagataaggcccaagaagaacatgagaaatatcacagtaattggagagcaatggctagtgattttaacctaccacctgtagtagcaaaagaaatagtagccagctgtgataaatgtcagctaaaaggggaagccatgcatggacaagtagactgtagcccaggaatatggcagctagattgtacacatttagaaggaaaagttatcttggtagcagttcatgtagccagtggatatatagaagcagaagtaattccagcagagacagggcaagaaacagcatacttcctcttaaaattagcaggaagatggccagtaaaaacagtacatacagacaatggcagcaatttcaccagtactacagttaaggccgcctgttggtgggcggggatcaagcaggaatttggcattccctacaatccccaaagtcaaggagtaatagaatctatgaataaagaattaaagaaaattataggacaggtaagagatcaggctgaacatcttaagacagcagtacaaatggcagtattcatccacaattttaaaagaaaaggggggattggggggtacagtgcaggggaaagaatagtagacataatagcaacagacatacaaactaaagaattacaaaaacaaattacaaaaattcaaaattttcgggtttattacagggacagcagagatccagtttggaaaggaccagcaaagctcctctggaaaggtgaaggggcagtagtaatacaagataatagtgacataaaagtagtgccaagaagaaaagcaaagatcatcagggattatggaaaacagatggcaggtgatgattgtgtggcaagtagacaggatgaggattaacacatggaaaagattagtaaaacaccatatgtatatttcaaggaaagctaaggactggttttatagacatcactatgaaagtactaatccaaaaataagttcagaagtacacatcccactaggggatgctaaattagtaataacaacatattggggtctgcatacaggagaaagagactggcatttgggtcagggagtctccatagaatggaggaaaaagagatatagcacacaagtagaccctgacctagcagaccaactaattcatctgcactattttgattgtttttcagaatctgctataagaaataccatattaggacgtatagttagtcctaggtgtgaatatcaagcaggacataacaaggtaggatctctacagtacttggcactagcagcattaataaaaccaaaacagataaagccacctttgcctagtgttaggaaactgacagaggacagatggaacaagccccagaagaccaagggccacagagggagccatacaatgaatggacactagagcttttagaggaacttaagagtgaagctgttagacattttcctaggatatggctccataacttaggacaacatatctatgaaacttacggggatacttgggcaggagtggaagccataataagaattctgcaacaactgctgtttatccatttcagaattgggtgtcgacatagcagaataggcgttactcgacagaggagagcaagaaatggagccagtagatcctagactagagccctggaagcatccaggaagtcagcctaaaactgcttgtaccaattgctattgtaaaaagtgttgctttcattgccaagtttgtttcatgacaaaagccttaggcatctcctatggcaggaagaagcggagacagcgacgaagagctcatcagaacagtcagactcatcaagcttctctatcaaagcagtaagtagtacatgtaatgcaacctataatagtagcaatagtagcattagtagtagcaataataatagcaatagttgtgtggtccatagtaatcatagaatataggaaaatattaagacaaagaaaaatagacaggttaattgatagactaatagaaagagcagaagacagtggcaatgagagtgaaggagaagtatcagcacttgtggagatgggggtggaaatggggcaccatgctccttgggatattgatgatctgtagtgctacagaaaaattgtgggtcacagtctattatggggtacctgtgtggaaggaagcaaccaccactctattttgtgcatcagatgctaaagcatatgatacagaggtacataatgtttgggccacacatgcctgtgtacccacagaccccaacccacaagaagtagtattggtaaatgtgacagaaaattttaacatgtggaaaaatgacatggtagaacagatgcatgaggatataatcagtttatgggatcaaagcctaaagccatgtgtaaaattaaccccactctgtgttagtttaaagtgcactgatttgaagaatgatactaataccaatagtagtagcgggagaatgataatggagaaaggagagataaaaaactgctctttcaatatcagcacaagcataagagataaggtgcagaaagaatatgcattcttttataaacttgatatagtaccaatagataataccagctataggttgataagttgtaacacctcagtcattacacaggcctgtccaaaggtatcctttgagccaattcccatacattattgtgccccggctggttttgcgattctaaaatgtaataataagacgttcaatggaacaggaccatgtacaaatgtcagcacagtacaatgtacacatggaatcaggccagtagtatcaactcaactgctgttaaatggcagtctagcagaagaagatgtagtaattagatctgccaatttcacagacaatgctaaaaccataatagtacagctgaacacatctgtagaaattaattgtacaagacccaacaacaatacaagaaaaagtatccgtatccagaggggaccagggagagcatttgttacaataggaaaaataggaaatatgagacaagcacattgtaacattagtagagcaaaatggaatgccactttaaaacagatagctagcaaattaagagaacaatttggaaataataaaacaataatctttaagcaatcctcaggaggggacccagaaattgtaacgcacagttttaattgtggaggggaatttttctactgtaattcaacacaactgtttaatagtacttggtttaatagtacttggagtactgaagggtcaaataacactgaaggaagtgacacaatcacactcccatgcagaataaaacaatttataaacatgtggcaggaagtaggaaaagcaatgtatgcccctcccatcagtggacaaattagatgttcatcaaatattactgggctgctattaacaagagatggtggtaataacaacaatgggtccgagatcttcagacctggaggaggcgatatgagggacaattggagaagtgaattatataaatataaagtagtaaaaattgaaccattaggagtagcacccaccaaggcaaagagaagagtggtgcagagagaaaaaagagcagtgggaataggagctttgttccttgggttcttgggagcagcaggaagcactatgggcgcagcgtcaatgacgctgacggtacaggccagacaattattgtctgatatagtgcagcagcagaacaatttgctgagggctattgaggcgcaacagcatctgttgcaactcacagtctggggcatcaaacagctccaggcaagaatcctggctgtggaaagatacctaaaggatcaacagctcctggggatttggggttgctctggaaaactcatttgcaccactgctgtgccttggaatgctagttggagtaataaatctctggaacagatttggaataacatgacctggatggagtgggacagagaaattaacaattacacaagcttaatacactccttaattgaagaatcgcaaaaccagcaagaaaagaatgaacaagaattattggaattagataaatgggcaagtttgtggaattggtttaacataacaaattggctgtggtatataaaattattcataatgatagtaggaggcttggtaggtttaagaatagtttttgctgtactttctatagtgaatagagttaggcagggatattcaccattatcgtttcagacccacctcccaatcccgaggggacccgacaggcccgaaggaatagaagaagaaggtggagagagagacagagacagatccattcgattagtgaacggatccttagcacttatctgggacgatctgcggagcctgtgcctcttcagctaccaccgcttgagagacttactcttgattgtaacgaggattgtggaacttctgggacgcagggggtgggaagccctcaaatattggtggaatctcctacagtattggagtcaggaactaaagaatagtgctgttaacttgctcaatgccacagccatagcagtagctgaggggacagatagggttatagaagtattacaagcagcttatagagctattcgccacatacctagaagaataagacagggcttggaaaggattttgctataagatgggtggcaagtggtcaaaaagtagtgtgattggatggcctgctgtaagggaaagaatgagacgagctgagccagcagcagatggggtgggagcagtatctcgagacctagaaaaacatggagcaatcacaagtagcaatacagcagctaacaatgctgcttgtgcctggctagaagcacaagaggaggaagaggtgggttttccagtcacacctcaggtacctttaagaccaatgacttacaaggcagctgtagatcttagccactttttaaaagaaaaggggggactggaagggctaattcactcccaaagaagacaagatatccttgatctgtggatctaccacacacaaggctacttccctgattggcagaactacacaccagggccaggggtcagatatccactgacctttggatggtgctacaagctagtaccagttgagccagataaggtagaagaggccaataaaggagagaacaccagcttgttacaccctgtgagcctgcatggaatggatgaccctgagagagaagtgttagagtggaggtttgacagccgcctagcatttcatcacgtggcccgagagctgcatccggagtacttcaagaactgctgacatcgagcttgctacaagggactttccgctggggactttccagggaggcgtggcctgggcgggactggggagtggcgagccctcagatgctgcatataagcagctgctttttgcctgtactgggtctctctggttagaccagatctgagcctgggagctctctggctaactagggaacccactgcttaagcctcaataaagcttgccttgagtgcttcaagtagtgtgtgcccgtctgttgtgtgactctggtaactagagatccctcagacccttttagtcagtgtggaaaatctctagcacccaggaggtagaggttgcagtgagccaagatcgcgccactgcattccagcctgggcaagaaaacaagactgtctaaaataataataataagttaagggtattaaatatatttatacatggaggtcataaaaatatatatatttgggctgggcgcagtggctcacacctgcgcccggccctttgggaggccgaggcaggtggatcacctgagtttgggagttccagaccagcctgaccaacatggagaaaccccttctctgtgtatttttagtagattttattttatgtgtattttattcacaggtatttctggaaaactgaaactgtttttcctctactctgataccacaagaatcatcagcacagaggaagacttctgtgatcaaatgtggtgggagagggaggttttcaccagcacatgagcagtcagttctgccgcagactcggcgggtgtccttcggttcagttccaacaccgcctgcctggagagaggtcagaccacagggtgagggctcagtccccaagacataaacacccaagacataaacacccaacaggtccaccccgcctgctgcccaggcagagccgattcaccaagacgggaattaggatagagaaagagtaagtcacacagagccggctgtgcgggagaacggagttctattatgactcaaatcagtctccccaagcattcggggatcagagtttttaaggataacttagtgtgtagggggccagtgagttggagatgaaagcgtagggagtcgaaggtgtccttttgcgccgagtcagttcctgggtgggggccacaagatcggatgagccagtttatcaatccgggggtgccagctgatccatggagtgcagggtctgcaaaatatctcaagcactgattgatcttaggttttacaatagtgatgttaccccaggaacaatttggggaaggtcagaatcttgtagcctgtagctgcatgactcctaaaccataatttcttttttgtttttttttttttatttttgagacagggtctcactctgtcacctaggctggagtgcagtggtgcaatcacagctcactgcagcctcaacgtcgtaagctcaagcgatcctcccacctcagcctgcctggtagctgagactacaagcgacgccccagttaatttttgtatttttggtagaggcagcgttttgccgtgtggccctggctggtctcgaactcctgggctcaagtgatccagcctcagcctcccaaagtgctgggacaaccggggccagtcactgcacctggccctaaaccataatttctaatcttttggctaatttgttagtcctacaaaggcagtctagtccccaggcaaaaagggggtttgtttcgggaaagggctgttactgtctttgtttcaaactataaactaagttcctcctaaacttagttcggcctacacccaggaatgaacaaggagagcttggaggttagaagcacgatggaattggttaggtcagatctctttcactgtctgagttataattttgcaatggtggttcaaagactgcccgcttctgacaccagtcgctgcattaatgaatcggccaacgcgcggggagaggcggtttgcgtattgggcgctcttccgcttcctcgctcactgactcgctgcgctcggtcgttcggctgcggcgagcggtatcagctcactcaaaggcggtaatacggttatccacagaatcaggggataacgcaggaaagaacatgtgagcaaaaggccagcaaaaggccaggaaccgtaaaaaggccgcgttgctggcgtttttccataggctccgcccccctgacgagcatcacaaaaatcgacgctcaagtcagaggtggcgaaacccgacaggactataaagataccaggcgtttccccctggaagctccctcgtgcgctctcctgttccgaccctgccgcttaccggatacctgtccgcctttctcccttcgggaagcgtggcgctttctcatagctcacgctgtaggtatctcagttcggtgtaggtcgttcgctccaagctgggctgtgtgcacgaaccccccgttcagcccgaccgctgcgccttatccggtaactatcgtcttgagtccaacccggtaagacacgacttatcgccactggcagcagccactggtaacaggattagcagagcgaggtatgtaggcggtgctacagagttcttgaagtggtggcctaactacggctacactagaagaacagtatttggtatctgcgctctgctgaagccagttaccttcggaaaaagagttggtagctcttgatccggcaaacaaaccaccgctggtagcggtggtttttttgtttgcaagcagcagattacgcgcagaaaaaaaggatctcaagaagatcctttgatcttttctacggggtctgacgctcagtggaacgaaaactcacgttaagggattttggtcatgagattatcaaaaaggatcttcacctagatccttttaaattaaaaatgaagttttaaatcaatctaaagtatatatgagtaaacttggtctgacagttaccaatgcttaatcagtgaggcacctatctcagcgatctgtctatttcgttcatccatagttgcctgactccccgtcgtgtagataactacgatacgggagggcttaccatctggccccagtgctgcaatgataccgcgagacccacgctcaccggctccagatttatcagcaataaaccagccagccggaagggccgagcgcagaagtggtcctgcaactttatccgcctccatccagtctattaattgttgccgggaagctagagtaagtagttcgccagttaatagtttgcgcaacgttgttgccattgctacaggcatcgtggtgtcacgctcgtcgtttggtatggcttcattcagctccggttcccaacgatcaaggcgagttacatgatcccccatgttgtgcaaaaaagcggttagctccttcggtcctccgatcgttgtcagaagtaagttggccgcagtgttatcactcatggttatggcagcactgcataattctcttactgtcatgccatccgtaagatgcttttctgtgactggtgagtactcaaccaagtcattctgagaatagtgtatgcggcgaccgagttgctcttgcccggcgtcaatacgggataataccgcgccacatagcagaactttaaaagtgctcatcattggaaaacgttcttcggggcgaaaactctcaaggatcttaccgctgttgagatccagttcgatgtaacccactcgtgcacccaactgatcttcagcatcttttactttcaccagcgtttctgggtgagcaaaaacaggaaggcaaaatgccgcaaaaaagggaataagggcgacacggaaatgttgaatactcatactcttcctttttcaatattattgaagcatttatcagggttattgtctcatgagcggatacatatttgaatgtatttagaaaaataaacaaataggggttccgcgcacatttccccgaaaagtgccacctgacgtctaagaaaccattattatcatgacattaacctataaaaataggcgtatcacgaggccctttcgtctcgcgcgtttcggtgatgacggtgaaaacctctgacacatgcagctcccggagacggtcacagcttgtctgtaagcggatgccgggagcagacaagcccgtcagggcgcgtcagcgggtgttggcgggtgtcggggctggcttaactatgcggcatcagagcagattgtactgagagtgcaccatatgcggtgtgaaataccgcacagatgcgtaaggagaaaataccgcatcaggcgccattcgccattcaggctgcgcaactgttgggaagggcgatcggtgcgggcctcttcgctattacgccaggggaggcagagattgcagtaagctgagatcgcagcactgcactccagcctgggcgacagagtaagactctgtctcaaaaataaaataaataaatcaatcagatattccaatcttttcctttatttatttatttattttctattttggaaacacagtccttccttattccagaattacacatatattctatttttctttatatgctccagttttttttagaccttcacctgaaatgtgtgtatacaaaatctaggccagtccagcagagcctaaaggtaaaaaataaaataataaaaaataaataaaatctagctcactccttcacatcaaaatggagatacagctgttagcattaaataccaaataacccatcttgtcctcaataattttaagcgcctctctccaccacatctaactcctgtcaaaggcatgtgccccttccgggcgctctgctgtgctgccaaccaactggcatgtggactctgcagggtccctaactgccaagccccacagtgtgccctgaggctgccccttccttctagcggctgcccccactcggctttgctttccctagtttcagttacttgcgttcagccaaggtctgaaactaggtgcgcacagagcggtaagactgcgagagaaagagaccagctttacagggggtttatcacagtgcaccctgacagtcgtcagcctcacagggggtttatcacattgcaccctgacagtcgtcagcctcacagggggtttatcacagtgcacccttacaatcattccatttgattcacaatttttttagtctctactgtgcctaacttgtaagttaaatttgatcagaggtgtgttcccagaggggaaaacagtatatacagggttcagtactatcgcatttcaggcctccacctgggtcttggaatgtgtcccccgaggggtgatgactacctcagttggatctccacaggtcacagtgacacaagataaccaagacacctcccaaggctaccacaatgggccgccctccacgtgcacatggccggaggaactgccatgtcggaggtgcaagcacacctgcgcatcagagtccttggtgtggagggagggaccagcgcagcttccagccatccacctgatgaacagaacctagggaaagccccagttctacttacaccaggaaaggc

SEQ ID NO: 385 - DNA, 10535 bp, Simian immunodeficiency virus
  source 1..10535: mol_type = unassigned DNA
gcatgcacattttaaaggcttttgctaaatatagccaaaagtccttctacaaattttctaagagttctgattcaaagcagtaacaggccttgtctcatcatgaactttggcatttcatctacagctaagtttatatcataaatagttctttacaggcagcaccaacttatacccttatagcatactttactgtgtgaaaattgcatctttcattaagcttactgtaaatttactggctgtcttccttgcaggtttctggaagggatttattacagtgcaagaagacatagaatcttagacatatacttagaaaaggaagaaggcatcataccagattggcaggattacacctcaggaccaggaattagatacccaaagacatttggctggctatggaaattagtccctgtaaatgtatcagatgaggcacaggaggatgaggagcattatttaatgcatccagctcaaacttcccagtgggatgacccttggggagaggttctagcatggaagtttgatccaactctggcctacacttatgaggcatatgttagatacccagaagagtttggaagcaagtcaggcctgtcagaggaagaggttagaagaaggctaaccgcaagaggccttcttaacatggctgacaagaaggaaactcgctgaaacagcagggactttccacaaggggatgttacggggaggtactggggaggagccggtcgggaacgcccactttcttgatgtataaatatcactgcatttcgctctgtattcagtcgctctgcggagaggctggcagattgagccctgggaggttctctccagcactagcaggtagagcctgggtgttccctgctagactctcaccagcacttggccggtgctgggcagagtgactccacgcttgcttgcttaaagccctcttcaataaagctgccattttagaagtaagctagtgtgtgttcccatctctcctagccgccgcctggtcaactcggtactcaataataagaagaccctggtctgttaggaccctttctgctttgggaaaccgaagcaggaaaatccctagcagattggcgcctgaacagggacttgaaggagagtgagagactcctgagtacggctgagtgaaggcagtaagggcggcaggaaccaaccacgacggagtgctcctataaaggcgcgggtcggtaccagacggcgtgaggagcgggagaggaagaggcctccggttgcaggtaagtgcaacacaaaaaagaaatagctgtcttttatccaggaaggggtaataagatagagtgggagatgggcgtgagaaactccgtcttgtcagggaagaaagcagatgaattagaaaaaattaggctacgacccaacggaaagaaaaagtacatgttgaagcatgtagtatgggcagcaaatgaattagatagatttggattagcagaaagcctgttggagaacaaagaaggatgtcaaaaaatactttcggtcttagctccattagtgccaacaggctcagaaaatttaaaaagcctttataatactgtctgcgtcatctggtgcattcacgcagaagagaaagtgaaacacactgaggaagcaaaacagatagtgcagagacacctagtggtggaaacaggaacaacagaaactatgccaaaaacaagtagaccaacagcaccatctagcggcagaggaggaaattacccagtacaacaaataggtggtaactatgtccacctgccattaagcccgagaacattaaatgcctgggtaaaattgatagaggaaaagaaatttggagcagaagtagtgccaggatttcaggcactgtcagaaggttgcaccccctatgacattaatcagatgttaaattgtgtgggagaccatcaagcggctatgcagattatcagagatattataaacgaggaggctgcagattgggacttgcagcacccacaaccagctccacaacaaggacaacttagggagccgtcaggatcagatattgcaggaacaactagttcagtagatgaacaaatccagtggatgtacagacaacagaaccccataccagtaggcaacatttacaggagatggatccaactggggttgcaaaaatgtgtcagaatgtataacccaacaaacattctagatgtaaaacaagggccaaaagagccatttcagagctatgtagacaggttctacaaaagtttaagagcagaacagacagatgcagcagtaaagaattggatgactcaaacactgctgattcaaaatgctaacccagattgcaagctagtgctgaaggggctgggtgtgaatcccaccctagaagaaatgctgacggcttgtcaaggagtaggggggccgggacagaaggctagattaatggcagaagccctgaaagaggccctcgcaccagtgccaatcccttttgcagcagcccaacagaggggaccaagaaagccaattaagtgttggaattgtgggaaagagggacactctgcaaggcaatgcagagccccaagaagacagggatgctggaaatgtggaaaaatggaccatgttatggccaaatgcccagacagacaggcgggttttttaggccttggtccatggggaaagaagccccgcaatttccccatggctcaagtgcatcaggggctgatgccaactgctcccccagaggacccagctgtggatctgctaaagaactacatgcagttgggcaagcagcagagagaaaagcagagagaaagcagagagaagccttacaaggaggtgacagaggatttgctgcacctcaattctctctttggaggagaccagtagtcactgctcatattgaaggacagcctgtagaagtattactggatacaggggctgatgattctattgtaacaggaatagagttaggtccacattataccccaaaaatagtaggaggaataggaggttttattaatactaaagaatacaaaaatgtagaaatagaagttttaggcaaaaggattaaagggacaatcatgacaggggacaccccgattaacatttttggtagaaatttgctaacagctctggggatgtctctaaattttcccatagctaaagtagagcctgtaaaagtcgccttaaagccaggaaaggatggaccaaaattgaagcagtggccattatcaaaagaaaagatagttgcattaagagaaatctgtgaaaagatggaaaaggatggtcagttggaggaagctcccccgaccaatccatacaacacccccacatttgctataaagaaaaaggataagaacaaatggagaatgctgatagattttagggaactaaatagggtcactcaggactttacggaagtccaattaggaataccacaccctgcaggactagcaaaaaggaaaagaattacagtactggatataggtgatgcatatttctccatacctctagatgaagaatttaggcagtacactgcctttactttaccatcagtaaataatgcagagccaggaaaacgatacatttataaggttctgcctcagggatggaaggggtcaccagccatcttccaatacactatgagacatgtgctagaacccttcaggaaggcaaatccagatgtgaccttagtccagtatatggatgacatcttaatagctagtgacaggacagacctggaacatgacagggtagttttacagtcaaaggaactcttgaatagcatagggttttctaccccagaagagaaattccaaaaagatcccccatttcaatggatggggtacgaattgtggccaacaaaatggaagttgcaaaagatagagttgccacaaagagagacctggacagtgaatgatatacagaagttagtaggagtattaaattgggcagctcaaatttatccaggtataaaaaccaaacatctctgtaggttaattagaggaaaaatgactctaacagaggaagttcagtggactgagatggcagaagcagaatatgaggaaaataaaataattctcagtcaggaacaagaaggatgttattaccaagaaggcaagccattagaagccacggtaataaagagtcaggacaatcagtggtcttataaaattcaccaagaagacaaaatactgaaagtaggaaaatttgcaaagataaagaatacacataccaatggagtgagactattagcacatgtaatacagaaaataggaaaggaagcaatagtgatctggggacaggtcccaaaattccacttaccagttgagaaggatgtatgggaacagtggtggacagactattggcaggtaacctggataccggaatgggattttatctcaacaccaccgctagtaagattagtcttcaatctagtgaaggaccctatagagggagaagaaacctattatacagatggatcatgtaataaacagtcaaaagaagggaaagcaggatatatcacagataggggcaaagacaaagtaaaagtgttagaacagactactaatcaacaagcagaattggaagcatttctcatggcattgacagactcagggccaaaggcaaatattatagtagattcacaatatgttatgggaataataacaggatgccctacagaatcagagagcaggctagttaatcaaataatagaagaaatgattaaaaagtcagaaatttatgtagcatgggtaccagcacacaaaggtataggaggaaaccaagaaatagaccacctagttagtcaagggattagacaagttctcttcttggaaaagatagagccagcacaagaagaacatgataaataccatagtaatgtaaaagaattggtattcaaatttggattacccagaatagtggccagacagatagtagacacctgtgataaatgtcatcagaaaggagaggctatacatgggcaggcaaattcagatctagggacttggcaaatggattgtacccatctagagggaaaaataatcatagttgcagtacatgtagctagtggattcatagaagcagaggtaattccacaagagacaggaagacagacagcactatttctgttaaaattggcaggcagatggcctattacacatctacacacagataatggtgctaactttgcttcgcaagaagtaaagatggttgcatggtgggcagggatagagcacacctttggggtaccatacaatccacagagtcagggagtagtggaagcaatgaatcaccacctgaaaaatcaaatagatagaatcagggaacaagcaaattcagtagaaaccatagtattaatggcagttcattgcatgaattttaaaagaaggggaggaataggggatatgactccagcagaaagattaattaacatgatcactacagaacaagagatacaatttcaacaatcaaaaaactcaaaatttaaaaattttcgggtctattacagagaaggcagagatcaactgtggaagggacccggtgagctattgtggaaaggggaaggagcagtcatcttaaaggtagggacagacattaaggtagtacccagaagaaaggctaaaattatcaaagattatggaggaggaaaagaggtggatagcagttcccacatggaggataccggagaggctagagaggtggcatagcctcataaaatatctgaaatataaaactaaagatctacaaaaggtttgctatgtgccccattttaaggtcggatgggcatggtggacctgcagcagagtaatcttcccactacaggaaggaagccatttagaagtacaagggtattggcatttgacaccagaaaaagggtggctcagtacttatgcagtgaggataacctggtactcaaagaacttttggacagatgtaacaccaaactatgcagacattttactgcatagcacttatttcccttgctttacagcgggagaagtgagaagggccatcaggggagaacaactgctgtcttgctgcaggttcccgagagctcataagtaccaggtaccaagcctacagtacttagcactgaaagtagtaagcgatgtcagatcccagggagagaatcccacctggaaacagtggagaagagacaataggagaggccttcgaatggctaaacagaacagtagaggagataaacagagaggcggtaaaccacctaccaagggagctaattttccaggtttggcaaaggtcttgggaatactggcatgatgaacaagggatgtcaccaagctatgtaaaatacagatacttgtgtttaatacaaaaggctttatttatgcattgcaagaaaggctgtagatgtctaggggaaggacatggggcagggggatggagaccaggacctcctcctcctccccctccaggactagcataaatggaagaaagacctccagaaaatgaaggaccacaaagggaaccatgggatgaatgggtagtggaggttctggaagaactgaaagaagaagctttaaaacattttgatcctcgcttgctaactgcacttggtaatcatatctataatagacatggagacacccttgagggagcaggagaactcattagaatcctccaacgagcgctcttcatgcatttcagaggcggatgcatccactccagaatcggccaacctgggggaggaaatcctctctcagctataccgccctctagaagcatgctataacacatgctattgtaaaaagtgttgctaccattgccagttttgttttcttaaaaaaggcttggggatatgttatgagcaatcacgaaagagaagaagaactccgaaaaaggctaaggctaatacatcttctgcatcaaacaagtaagtatgggatgtcttgggaatcagctgcttatcgccatcttgcttttaagtgtctatgggatctattgtactctatatgtcacagtcttttatggtgtaccagcttggaggaatgcgacaattcccctcttttgtgcaaccaagaatagggatacttggggaacaactcagtgcctaccagataatggtgattattcagaagtggcccttaatgttacagaaagctttgatgcctggaataatacagtcacagaacaggcaatagaggatgtatggcaactctttgagacctcaataaagccttgtgtaaaattatccccattatgcattactatgagatgcaataaaagtgagacagatagatggggattgacaaaatcaataacaacaacagcatcaacaacatcaacgacagcatcagcaaaagtagacatggtcaatgagactagttcttgtatagcccaggataattgcacaggcttggaacaagagcaaatgataagctgtaaattcaacatgacagggttaaaaagagacaagaaaaaagagtacaatgaaacttggtactctgcagatttggtatgtgaacaagggaataacactggtaatgaaagtagatgttacatgaaccactgtaacacttctgttatccaagagtcttgtgacaaacattattgggatgctattagatttaggtattgtgcacctccaggttatgctttgcttagatgtaatgacacaaattattcaggctttatgcctaaatgttctaaggtggtggtctcttcatgcacaaggatgatggagacacagacttctacttggtttggctttaatggaactagagcagaaaatagaacttatatttactggcatggtagggataataggactataattagtttaaataagtattataatctaacaatgaaatgtagaagaccaggaaataagacagttttaccagtcaccattatgtctggattggttttccactcacaaccaatcaatgataggccaaagcaggcatggtgttggtttggaggaaaatggaaggatgcaataaaagaggtgaagcagaccattgtcaaacatcccaggtatactggaactaacaatactgataaaatcaatttgacggctcctggaggaggagatccggaagttaccttcatgtggacaaattgcagaggagagttcctctactgtaaaatgaattggtttctaaattgggtagaagataggaatacagctaaccagaagccaaaggaacagcataaaaggaattacgtgccatgtcatattagacaaataatcaacacttggcataaagtaggcaaaaatgtttatttgcctccaagagagggagacctcacgtgtaactccacagtgaccagtctcatagcaaacatagattggattgatggaaaccaaactaatatcaccatgagtgcagaggtggcagaactgtatcgattggaattgggagattataaattagtagagatcactccaattggcttggcccccacagatgtgaagaggtacactactggtggcacctcaagaaataaaagaggggtctttgtgctagggttcttgggttttctcgcaacggcaggttctgcaatgggcgcggcgtcgttgacgctgaccgctcagtcccgaactttattggctgggatagtgcagcaacagcaacagctgttggacgtggtcaagagacaacaagaattgttgcgactgaccgtctggggaacaaagaacctccagactagggtcactgccatcgagaagtacttaaaggaccaggcgcagctgaatgcttggggatgtgcgtttagacaagtctgccacactactgtaccatggccaaatgcaagtctaacaccaaagtggaacaatgagacttggcaagagtgggagcgaaaggttgacttcttggaagaaaatataacagccctcctagaggaggcacaaattcaacaagagaagaacatgtatgaattacaaaagttgaatagctgggatgtgtttggcaattggtttgaccttgcttcttggataaagtatatacaatatggagtttatatagttgtaggagtaatactgttaagaatagtgatctatatagtacaaatgctagctaagttaaggcaggggtataggccagtgttctcttccccaccctcttatttccagcagacccatatccaacaggacccggcactgccaaccagagaaggcaaagaaagagacggtggagaaggcggtggcaacagctcctggccttggcagatagaatatattcatttcctgatccgccaactgatacgcctcttgacttggctattcagcaactgcagaaccttgctatcgagagtataccagatcctccaaccaatactccagaggctctctgcgaccctacagaggattcgagaagtcctcaggactgaactgacctacctacaatatgggtggagctatttccatgaggcggtccaggccgtctggagatctgcgacagagactcttgcgggcgcgtggggagacttatgggagactcttaggagaggtggaagatggatactcgcaatccccaggaggattagacaagggcttgagctcactctcttgtgagggacagaaatacaatcagggacagtatatgaatactccatggagaaacccagctgaagagagagaaaaattagcatacagaaaacaaaatatggatgatatagatgagtaagatgatgacttggtaggggtatcagtgaggccaaaagttcccctaagaacaatgagttacaaattggcaatagacatgtctcattttataaaagaaaaggggggactggaagggatttattacagtgcaagaagacatagaatcttagacatatacttagaaaaggaagaaggcatcataccagattggcaggattacacctcaggaccaggaattagatacccaaagacatttggctggctatggaaattagtccctgtaaatgtatcagatgaggcacaggaggatgaggagcattatttaatgcatccagctcaaacttcccagtgggatgacccttggggagaggttctagcatggaagtttgatccaactctggcctacacttatgaggcatatgttagatacccagaagagtttggaagcaagtcaggcctgtcagaggaagaggttagaagaaggctaaccgcaagaggccttcttaacatggctgacaagaaggaaactcgctgaaacagcagggactttccacaaggggatgttacggggaggtactggggaggagccggtcgggaacgcccactttcttgatgtataaatatcactgcatttcgctctgtattcagtcgctctgcggagaggctggcagattgagccctgggaggttctctccagcactagcaggtagagcctgggtgttccctgctagactctcaccagcacttggccggtgctgggcagagtgactccacgcttgcttgcttaaagccctcttcaataaagctgccattttagaagtaagctagtgtgtgttcccatctctcctagccgccgcctggtcaactcggtactcaataataagaagaccctggtctgttaggaccctttctgctttgggaaaccgaagcaggaaaatccctagca

SEQ ID NO: 386 - DNA, 9713 bp, Human immunodeficiency virus 2
  source 1..9713: mol_type = unassigned DNA
agtcgctctgcggagaggctggcagattgagccctgggaggttctctccagcactagcaggtagagcctgggtgttccctgctagactctcaccggtgcttggccggcactgggcagacggctccacgcttgcttgcttaaaagacctcttaataaagctgccagttagaagcaagttaagtgtgtgttcccatctctcctagtcgccgcctggtcattcggtgttcatctgaataacaagaccctggtctgttaggaccctttctgctttgggaaaccaaagcaggaaaatccctagcaggttggcgcccgaacagggacttagagaagactgaaaagccttggaacacggctgagtgaaggcagtaagggcggcaggaacaaaccacgacggagtgctcctagaaaggcgcaggccaaggtaccaaaggcggcgtgtggagcgggagtaaagaggcctccgggtgaaggtaagtacctacaccaaaaaattgtagccaggaagggcttgttatcctacctttagacaggtagaagattgtgggagatgggcgcgagaaactccgtcttgaaagggaaaaaagcagacgaattagaaacaattaggttacggcccggcggaaagaaaaaatacaggctaaagcatattgtgtgggcagcgaatgaattggacagattcggattagcagagagcctgttggagtcaaaagaaggttgccaaagaattcttacagttttaggtccattagtaccgacaggttcagaaaatttaaaaagcctttttaatactgtctgcgtcatttggtgcatacacgcagaagagaaagtgaaagatactgaaggagcaaaacaaatagtacagagacatctagcggcagaaacaggaactgcagagaaaatgccaaatacaagtagaccaacagcaccacctagcgggaagggaggaaacttccccgtacaacaagtaggcggcaattatacccatgtgccgctgagtcctcgaaccctaaatgcttgggtaaaattagtagaggaaaagaagttcggggcagaggtagtgccaggatttcaggcactctcagaaggctgcacgccctatgatatcaaccaaatgcttaattgtgtgggcgaccatcaagcagctatgcaaataatcagggagatcgttaatgaagaagcagcagattgggatgtgcaacatccaataccaggtcccttaccagcggggcagcttagagaaccaagagggtctgacatagcagggacaacaagcacagtagatgaacagatccagtggatgtttaggccacaaaatcccgtaccagtgggaaacatctataggagatggatccagataggactgcagaagtgcgtcaggatgtacaacccgaccaacatcctagacataaaacaaggaccaaaggaaccattccaaagttatgtagatagattctacaaaagcttgagggcagaacaaacagatccagcagtgaagaattggatgacccagacactactagtacagaatgccaacccagactgtaaattagtactaaaaggactagggatgaatcctaccttagaagagatgctaaccgcctgccaaggggtaggtgggccaggccagaaagctagactaatggcagaagccttaaaagaggccttgacaccagcccctatcccatttgcagcagcccagcagaaaaggacaattaaatgctggaattgtggaaaggaaggacactcggcaagacaatgccgagcacctagaagacagggctgctggaagtgtggtaaaccaggacatgtcatagcaaattgcccagatagacaggtgggttttttagggatgggcccccggggaaagaagccccgcaacttccccgtggcccaagtcccgcaggggctaacaccaacagcacccccagtagatccagcagtggacctactggagaattatatgcagcaaggaaaaagacaaagagaacagagagagagaccatacaaagaagtgacagaggacttactgcacctcgagcagggagaggcaccatgcagagagacgacagaggacttgctgcacctcaattctctcttttgaaaagaccagtagtcacggcatacgtcgagggccagccagtagaagttctgctagacacgggggctgacgactcaatagtagcagggatagagttagggagcaattatagtccaaagatagtaggaggaatagggggattcataaataccaaggaatataaaaatgtaaaaatagaagttttaggtaaaaaggtaagggccaccataatgacaggtgacaccccaatcaacatttttggcagaaatattctgacagccttaggcatgtcattaaatttaccagtcgccaaaatagaaccaataaaaataatgttaaagccaggaaaagatggaccaaaactgaggcaatggcccttaacaaaagaaaaaatagaggcactaaaagaaatctgtgaaaaaatggaaagagaaggccagctagaggaagcgcctccaactaatccttataacacccccacatttgcaatcaagaaaaaggacaaaaataaatggaggatgctaatagattttagagaactaaacaaggtaactcaagatttcacagaaattcagttaggaattccacacccagcaggattggccaagaaaaaaagaattactgtactagatataggggatgcttacttttccataccactacatgaagactttagacagtatactgcatttactttaccatcaataaacaatgcagaaccaggaaaaagatatatatataaggtcctgcctcagggatggaaggggtcaccagcaatttttcaatacacaatgaggcaggtcttagaaccattcagaaaagcaaacctagatgtcattatcattcagtacatggatgatatcctaatagctagtgacaggacagatctagaacatgacaaggtggtcctgcagctaaaggaacttctaaataacctaggattttctaccccagatgagaagttccaaaaggaccctccataccactggatgggctatgaactgtggccaactaagtggaagctgcagaagatacagttgccccaaaaagatgtatggacagtaaatgacatccaaaagttagtgggtgtcttaaactgggcagcacaaatctacccagggataaaaaccagacacttatgtaagctaattagaggaaaaatgacactcacagaagaagtacagtggacagaactagcagaggcggagttagaagagaacaagattatcttaagccaggagcaagagggacactattaccaagaagaaaaagagttagaagcaacagtccaaaaggatcaagacaatcagtggacatataaagtacaccagggagagaaaattctaaaagtagggaaatatgcaaagataaaaaatacccataccaatggggtcagattgttagcacaagtagttcaaaagataggaaaagaagcactaatcatttggggacgaataccaaaatttcacctaccagtagaaagagagacatgggaacagtggtgggatgactactggcaggtgacatggatccctgactgggacttcgtatctaccccgccgctggtcagactagcatttaacctggtaaaagatcctataccaagaacagagactttctacacagatggatcctgcaataggcaatcaaaggaaggaaaagcaggatatgtaacagatagagggagagacaaggtaaggatgctagaacaaactaccaatcagcaagcagaattagaagcctttgcaatggcactaacagactcaggtccaaaagccaatattatagtagactcacagtatgtaatggggatagtagcaggccagccaacagaatcagagagtagaatagtaaatcaaatcatagaggagatgataaaaaaggaagcaatctatgttgcatgggtcccagcccataaaggcataggagggaatcaggaggtagatcagttagtaagtcagggcatcagacaagtgttgttcctggaaaaaatagagcccgctcaggaagaacatgagaaataccatagcaatgtaaaagaactatcccataaatttggattgcccaaattagtagcaagacaaatagtaaacacatgtgcccaatgtcaacagaaaggggaggctatacatgggcaagtagatgcagaattaggcacttggcaaatggactgcacacacttagaaggaaagatcattatagtagcagtacatgttgcaagtggattcatagaagcagaagtcatcccacaggaatcaggaaggcagacagcactcttcctattaaaactggccagtaggtggccaataacacacttgcacacagataatggtgccaacttcacttcacaggaagtaaaaatggtagcatggtgggtaggtatagaacaatctttcggagtaccttacaatccacaaagccaaggagtagtagaagcaatgaatcaccacctaaaaaatcagataagtagaattagagaacaggcaaatacagtagaaacaatagtactgatggcaacacactgcatgaattttaaaagaaggggaggaataggggatatgaccccagcagaaagactaatcaatatgatcaccacagaacaagaaatacaattcctccacgccaaaaattcaaaattaaaaaattttcgggtctatttcagagaaggcagagatcagctgtggaaaggacccggggaactactgtggaagggagacggagcagtcatagtcaaggtagggacagacataaaagtagtaccaaggaggaaagccaagatcatcaaagactatggaggaaggcaagaactggatagtggttcccacttggagggtgccagggaggatggagaaatggcatagccttgtcaaatatctaaaatacagaacaaaagatctagaagacgtgtgctatgttccccaccataaagtaggatgggcatggtggacttgcagcagggtaatattcccattaaagggaaacagtcatctagaaatacaggcatattggaacctaacgccagaaaaaggatggctctcctcttattcagtaagaatgacttggtatacggaaaggttctggacagatgttaccccagactgtgcagactccctaatacatagcacttatttctcttgctttacagcaggtgaagtaagaagagccatcagaggggaaaagttattgtcctgctgcaattatccccaagcccatagagcccaggtaccgtcactccaatttttggccttagtggtagtgcagcaaaatgacagaccccagagaaacggtacccccaggaaacagtggcgaagagactatcgaagaggccttcaattggctagacaggacggtagaagccataaacagagaggcagtgaatcacctgccccgagagcttattttccaggtgtggcagaggtcctggagatactggcatgatgaacaagggatgtcacaaagttacacaaagtatagatatttgtgcttaatacagaaggctatgttcacacattgtaagagagggtgcacttgcctggggggaggacatgggccaggagggtggagaccaggacctccccctcctccccctccaggtctagtctaatgactgaagcaccaacagagtttcccccggaggatgggaccccaccgagggaaccaggggatgagtggataatagaaatcctgagaaaaataaagaaagaagctttaaagcattttgaccctcgcttgctaactgctcttggcaactatatccatactagacatggagacacccttgaaggcgccagagagctcattaatgtcctacaacgagccctcttcatgcacttcagagcgggatgtaggctctcaagaattggccaaacagggggaagaactcctttcccagctacatcgacccctagaaccatgcaataacaaatgctattgtaaaggatgctgcttccactgccagctgtgttttttaaacaaggggctcgggatatgttatgaccggaagggcagacgaagaagaactccgaagaaaactaaggctcattcatcttctgcatcagacaagtgagtatgatgggtggtagaaatcagctgcttgttgccattttgctaactagtacttgcttgatatattgcaccaattatgtgactgttttctatggcatacccgcgtggagaaatgcatccattcccctcttttgtgcaaccaagaatagggatacttggggaaccatacagtgcttgccagacaatgatgattatcaggagataactttgaatgtgacagaggctttcgatgcatgggataatacagtaacagaacaagcaatagaagatgtctggaatctatttgagacatcaataaaaccatgtgtcaaattaacgcctttatgtgtagcaatgagatgtaacaacacagatgcaaggaacacaaccacacccacaacagcatccccgcgtacaataaaacccgtgacagagataagtgagaattcctcatgcatacgcgcaaacaactgctcaggattgggagaagaagaggtggtcaattgtcaattcaatatgacaggattagagagagataagaaaaagcaatatagtgagacatggtactcgaaggatgtagtttgtgaaggaaatggcaccacagatacatgttacatgaaccattgcaacacatcggtcatcacagagtcatgtgacaagcactattgggatgctatgaggtttagatactgtgcaccaccaggttttgccctactaagatgcaatgataccaattattcaggctttgcgcccaattgctctaaggtagtagctgctacatgcaccagaatgatggaaacgcaaacttctacatggtttggctttaatggcactagagcagaaaatagaacatttatctattggcatggtagggataacagaactatcatcagcttaaacaaatattataatctcactatacattgtaagaggccaggaaataagacagtggtaccaataacacttatgtcagggttaaggtttcactcccagccggtcatcaataaaagacccagacaagcatggtgttggttcaaaggtgaatggaagggagccatgcaggaggtgaaggaaacccttgcaaaacatcccaggtataaaggaaccaatgaaacaaagaatattaactttacagcaccaggaaagggctcagacccagaggtggcatacatgtggactaactgcagaggagaatttctctactgcaacatgacttggttcctcaattggatagaaaataagacacaccgcaattatgtaccgtgccatataagacaaataattaacacctggcataaggtagggaaaaatgtatatttgcctcccagggaaggggagttgacctgcaactcaacagtaactagcataattgctaacattgatgcaaatggaaataatacaaatattacctttagtgcagaggtggcagaactataccgattagagttgggagattataaattggtagaaataacaccaattggcttcgcacctacagcagaaaaaagatactcctctactccaatgaggaacaagagaggtgtgttcgtgctagggttcttgggttttctcgcaacagcaggctctgcaatgggcgcggcgtccttaacgctgtcggctcagtctcggactttactggccgggatagtgcagcaacagcaacagctgttggacgtggtcaagagacaacaggaaatgttgcgactgaccgtctggggaacaaaaaatctccaggcaagagtcactgctatcgagaagtacttaaaggaccaggcgcaactaaattcatggggatgtgcatttagacaagtctgccacactactgtaccatgggtaaatgataccttaacgcctgagtggaacaatatgacgtggcaagaatgggaaggcaaaatccgcgacctggaggcaaatatcagtcaacaattagaacaagcacaaattcagcaagagaagaatatgtatgaactacaaaagttaaatagctgggatgtttttggtaactggtttgacttaacctcctggatcaagtatattcaatatggagtttatataataataggaatagtagttcttagaatagtaatatatatagtacagatgttaagtagacttagaaagggctataggcctgttttctcttccccccccggttacctccaacagatccatatccacaaggactgggaacagccagccagagaagaaacagaagaagacgttggaaacaacgttggagacagctcgtggccttggccgataagatatatacatttcctgatccaccagctgattcgcctcttggccggactatacaacatctgcaggaacttactatccaggatctccctgaccctccgaccagttttccagagtcttcagagggcactgacagcaatcagagactggctaagaactgacgcagcctacttgcagtatgggtgcgagtggatccaaggagcgttccaggccttcgcaagggctacgagagagactcttgcgggcacgtggagagacttgtggggggcactgcagcggatcgggaggggaatacttgcagtcccaagaagaatcaggcagggagcagagatcgccctcctatgagggacagcggtatcagcagggagactttatgaataccccatggagaaccccagcaaaagaaggggagaaagaattgtacaagcaacaaaatagagatgatgtagattcggatgatgatgacctagtaggggtctctgtcacaccaagagtaccactaagagaattgacacatagattagcaatagatgtgtcacattttataaaagaaaaagggggactggaagggatgtattacagtgagagaagacatagaatcttagacatataccttgaaaaggaagaagggataattgcagattggcagaactatactcatgggccaggaataagatacccaatgttctttgggtggctatggaagctagtaccagtagatgtcacacgacaggaggaggacgatgggactcactgtttactacacccagcacaaacaagcaggtttgatgacccgcatggggaaacactgatatggaagtttgaccccacgctggctcatgattacaaggcttttatcctgcacccagaggaatttgggcataagtcaggcctgccagaagaagactggaaggcaagactgaaagcaagagggataccatttagttagagacaggaacagctatatttggccagggcaggaaataactactgaaaacagctgagactgcagggactttccgaaggggctgtaaccaggggagggacatgggaggagccggtggggaacgccctcatactttctgtataaagatacccgctgcttgcattgtacttcagtcgctctgcggagaggctggcagattgagccctgggaggttctctccagcactagcaggtagagcctgggtgttccctgctagactctcaccggtgcttggccggcactgggcagacggctccacgcttgcttgcttaaaagacctcttaataaagctgccagttagaagcaagttaagtgtgtgttcccatctctcctagtcgccgcctggtc

SEQ ID NO: 387 - DNA, 11878 bp, synthetic construct
  misc_feature 1..11878: note = Description of Artificial Sequence: Synthetic polynucleotide
  source 1..11878: mol_type = other DNA
gcctcactgattaagcattggtaactgtcagaccaagtttactcatatatactttagattgatttaaaacttcatttttaatttaaaaggatctaggtgaagatcctttttgataatctcatgaccaaaatcccttaacgtgagttttcgttccactgagcgtcagaccccgtagaaaagatcaaaggatcttcttgagatcctttttttctgcgcgtaatctgctgcttgcaaacaaaaaaaccaccgctaccagcggtggtttgtttgccggatcaagagctaccaactctttttccgaaggtaactggcttcagcagagcgcagataccaaatactgttcttctagtgtagccgtagttaggccaccacttcaagaactctgtagcaccgcctacatacctcgctctgctaatcctgttaccagtggctgctgccagtggcgataagtcgtgtcttaccgggttggactcaagacgatagttaccggataaggcgcagcggtcgggctgaacggggggttcgtgcacacagcccagcttggagcgaacgacctacaccgaactgagatacctacagcgtgagctatgagaaagcgccacgcttcccgaagggagaaaggcggacaggtatccggtaagcggcagggtcggaacaggagagcgcacgagggagcttccagggggaaacgcctggtatctttatagtcctgtcgggtttcgccacctctgacttgagcgtcgatttttgtgatgctcgtcaggggggcggagcctatggaaaaacgccagcaacgcggcctttttacggttcctggccttttgctggccttttgctcacatgttctttcctgcgttatcccctgattctgtggataaccgtattaccgcctttgagtgagctgataccgctcgccgcagccgaacgaccgagcgcagcgagtcagtgagcgaggaagcggaagagcgcccaatacgcaaaccgcctctccccgcgcgttggccgattcattaatgcagctggcacgacaggtttcccgactggaaagcgggcagtgagcgcaacgcaattaatgtgagttagctcactcattaggcaccccaggctttacactttatgcttccggctcgtatgttgtgtggaattgtgagcggataacaatttcacacaggaaacagctatgaccatgattacgccaagctatttaggtgacactatagaatactcaagcttggggggatcctctagagtcgacctgcaggcatgctatttgatgaattaactacacttaaaataatacaattattattaaatttttttttgatttatttattaatttttaaacttaatcatttgtatttgggaggaattatatatatctttataattattttatttttttttatttttttatttttttattattattatttttttttattttttttttttactgtatcaaagaaaaacctttaaaaaaaaaattataatttccccatcttactatatttttaatacatacgttttaaggaattaaattagacaaaagctatattatgctttacatataattagaatttataaacgtttggttattagatatttcatgtctcagtaaagtctttcaatacatatgtaaaaaaatatatatgaatacacataagttgttaatatattttatatgcataaatgtataaatatatatatatatatatatatatgtatgtatgtatatgtgtgtatatgaaattatttcaatgtttaattttttaaattttaatttttttttttttttttttttttattatgtatattgatctttattatttaaatattacttttttcgttttttcttctttttattatttttttttttttttatattttatacaaatggtaattcaaataaaaggtataaatttatatttaattttcttttatggataaataaaagaaaaatataaatatataaaaatataaaaatatatatatgtatattggggtgatgataaaatgaaagataatatatatatatatatatctttatttttttttttttgtagaccccattgtgagtacataaatatattatataactcgggagcatcagtcatggaattcttatttctttttcttttttgcctggccggcctttttcgtggccgccggccttttgtcgcctcccagctgagacaggtcgatccgtgtctcgtacaggccggtgatgctctggtggatcagggtggcgtccagcacctctttggtgctggtgtacctcttccggtcgatggtggtgtcaaagtacttgaaggcggcaggggctcccagattggtcagggtaaacaggtggatgatattctcggcctgctctctgatgggcttatcccggtgcttgttgtaggcggacagcactttgtccagattagcgtcggccaggatcactctcttggagaactcgctgatctgctcgatgatctcgtccaggtagtgcttgtgctgttccacaaacagctgtttctgctcattatcctcgggggagcccttcagcttctcatagtggctggccaggtacaggaagttcacatatttggagggcagggccagttcgtttcccttctgcagttcgccggcagaggccagcattctcttccggccgttttccagctcgaacagggagtacttaggcagcttgatgatcaggtcctttttcacttctttgtagcccttggcttccagaaagtcgatgggattcttctcgaagctgcttctttccatgatggtgatccccagcagctctttcacactcttcagtttcttggacttgcccttttccactttggccaccaccagcacagaataggccacggtggggctgtcgaagccgccgtacttcttagggtcccagtccttctttctggcgatcagcttatcgctgttcctcttgggcaggatagactctttgctgaagccgcctgtctgcacctcggtctttttcacgatattcacttggggcatgctcagcactttccgcacggtggcaaaatcccggcccttatcccacacgatctccccggtttcgccgtttgtctcgatcagaggccgcttccggatctcgccgttggccagggtaatctcggtcttgaaaaagttcatgatgttgctgtagaagaagtacttggcggtagccttgccgatttcctgctcgctcttggcgatcatcttccgcacgtcgtacaccttgtagtcgccgtacacgaactcgctttccagcttagggtactttttgatcagggcggttcccacgacggcgttcaggtaggcgtcgtgggcgtggtggtagttgttgatctcgcgcactttgtaaaactggaaatccttccggaaatcggacaccagcttggacttcagggtgatcactttcacttcccggatcagcttgtcattctcgtcgtacttagtgttcatccgggagtccaggatctgtgccacgtgctttgtgatctgccgggtttccaccagctgtctcttgatgaagccggccttatccagttcgctcaggccgcctctctcggccttggtcagattgtcgaactttctctgggtaatcagcttggcgttcagcagctgccgccagtagttcttcatcttcttcacgacctcttcggagggcacgttgtcgctcttgccccggttcttgtcgcttctggtcagcaccttgttgtcgatggagtcgtccttcagaaagctctgaggcacgatatggtccacatcgtagtcggacagccggttgatgtccagttcctggtccacgtacatatcccgcccattctgcaggtagtacaggtacagcttctcgttctgcagctgggtgttttccacggggtgttctttcaggatctggctgcccagctctttgatgccctcttcgatccgcttcattctctcgcggctgttcttctgtcccttctgggtggtctggttctctctggccatttcgatcacgatgttctcgggcttgtgccggcccatcactttcacgagctcgtccaccaccttcactgtctgcaggatgcccttcttaatggcggggctgccggccagattggcaatgtgctcgtgcaggctatcgccctggccggacacctgggctttctggatgtcctctttaaaggtcaggctgtcgtcgtggatcagctgcatgaagtttctgttggcgaagccgtcggacttcaggaaatccaggattgtcttgccggactgcttgtcccggatgccgttgatcagcttccggctcagcctgccccagccggtgtatctccgccgcttcagctgcttcatcactttgtcgtcgaacaggtgggcataggttttcagccgttcctcgatcatctctctgtcctcaaacagtgtcagggtcagcacgatatcttccagaatgtcctcgttttcctcattgtccaggaagtccttgtccttgataattttcagcagatcgtggtatgtgcccagggaggcgttgaaccgatcttccacgccggagatttccacggagtcgaagcactcgattttcttgaagtagtcctctttcagctgcttcacggtcactttccggttggtcttgaacagcaggtccacgatggcctttttctgctcgccgctcaggaaggcgggctttctcattccctcggtcacgtatttcactttggtcagctcgttatacacggtgaagtactcgtacagcaggctgtgcttgggcagcaccttctcgttgggcaggttcttatcgaagttggtcatccgctcgatgaagctctgggcggaagcgcccttgtccaccacttcctcgaagttccagggggtgatggtttcctcgctctttctggtcatccaggcgaatctgctgtttcccctggccagagggcccacgtagtaggggatgcggaaggtcaggatcttctcgatcttttcccggttgtccttcaggaatgggtaaaaatcttcctgccgccgcagaatggcgtgcagctctcccaggtggatctggtgggggatgctgccgttgtcgaaggtccgctgcttccgcagcaggtcctctctgttcagcttcacgagcagttcctcggtgccgtccatcttttccaggatgggcttgatgaacttgtagaactcttcctggctggctccgccgtcaatgtagccggcgtagccgttcttgctctggtcgaagaaaatctctttgtacttctcaggcagctgctgccgcacgagagctttcagcagggtcaggtcctggtggtgctcgtcgtatctcttgatcatagaggcgctcaggggggccttggtgatctcggtgttcactctcaggatgtcgctcagcaggatggcgtcggacaggttcttggcggccagaaacaggtcggcgtactggtcgccgatctgggccagcaggttgtccaggtcgtcgtcgtaggtgtccttgctcagctgcagtttggcatcctcggccaggtcgaagttgctcttgaagttgggggtcaggcccaggctcagggcaatcaggtttccgaacaggccattcttcttctcgccgggcagctgggcgatcagattttccagccgtctgctcttgctcagtctggcagacaggatggccttggcgtccacgccgctggcgttgatggggttttcctcgaacagctggttgtaggtctgcaccagctggatgaacagcttgtccacgtcgctgttgtcggggttcaggtcgccctcgatcaggaagtggccccggaacttgatcatgtgggccagggccagatagatcagccgcaggtcggccttgtcggtgctgtccaccagtttctttctcaggtggtagatggtggggtacttctcgtggtaggccacctcgtccacgatgttgccgaagatggggtgccgctcgtgcttcttatcctcttccaccaggaaggactcttccagtctgtggaagaagctgtcgtccaccttggccatctcgttgctgaagatctcttgcagatagcagatccggttcttccgtctggtgtatcttcttctggcggttctcttcagccgggtggcctcggctgtttcgccgctgtcgaacagcagggctccgatcaggttcttcttgatgctgtgccggtcggtgttgcccagcaccttgaatttcttgctgggcaccttgtactcgtcggtgatcacggcccagcccacagagttggtgccgatgtccaggccgatgctgtacttcttgtcggctgctgggactccgtggataccgaccttccgcttcttctttggggccatcttatcgtcatcgtctttgtaatcaatatcatgatccttgtagtctccgtcgtggtccttatagtccatttttctcgagggatcctgatatatttctattaggtatttattattataaaatataaatcttgaatgataataaataaaatattagttattccttttctagtttaaaatatacatattataaatatatatatatatatatatatttttattgtgacaagaatatataattataaattatattatttatttttgtatttttttttttttttttttttttttctttttttgttttatttttctttttttttataaatattatttttttcttttatcatgcacattggaataatacattaatatatatatatatattatattatacatatattgaataatgtttataaaaaatgcataacttatatgaatataattttttttaaatatgacaaaaagaaaaaaaaaaaaaaccaaaaaaaattaaaattgaaatgaaatatataaatatattatttatatatattatacattgtttaatactactacatgtatatatatatattatatatatatatatatatcaattttttcaaaaataaattaatataaaaagaggggaaaaaaaaaaaaaaaaaaaaaaaaagataattaagtaagcatttaaaaatatataaattgataatatataaaattaatcacatataaaagcttataaacactaggttagctaattcgcttgtaagaggtactctcgtttatgcaaaactatttgatatagcattttaacaagtacacatatatatatgtaatatatatactatatatatctattgcatgtgtactaagcatgtgcatggcatcccctttttctcgtgtttaaaacagtttgtatgataaaatataaaggatttgaaaaagagaaaaaaatatatgatctcatcctatatagcgccataatttttatttgggttgaataaaattttctactaaatttaggtgtaagtaaaataatggaatatatataagtacaataaaaaagtgcataaattaaaaaatttttataataaatattttttttaaaaaagtcaataataatattaaatatatataacacaggattatatatgttcactacaattttttatattataatataaattcttttcaattttcattttattttacatacactttccttttttgtcactatattttaatattcacatatttagtttaaatactggctatttctttctacatttgctagtaacaattgtgtagtgcttaaatatatacacacacctaaaacttacaaagtatcctaggaccatggccaagcctttgtctcaagaagaatccaccctcattgaaagagcaacggctacaatcaacagcatccccatctctgaagactacagcgtcgccagcgcagctctctctagcgacggccgcatcttcactggtgtcaatgtatatcattttactgggggaccttgtgcagaactcgtggtgctgggcactgctgctgctgcggcagctggcaacctgacttgtatcgtcgcgatcggaaatgagaacaggggcatcttgagcccctgcggacggtgccgacaggtgcttctcgatctgcatcctgggatcaaagccatagtgaaggacagtgatggacagccgacggcagttgggattcgtgaattgctgccctctggttatgtgtgggagggctaaccgcgggtaccccattaaatttatttaataatagattaaaaatattataaaaataaaaacataaacacagaaattacaaaaaaaatacatatgaattttttttttgtaatcttccttataaatatagaataatgaatcatataaaacatatcattattcatttatttacatttaaaattattgtttcagtatctttaatttattatgtatatataaaaataacttacaattttattaataaacaatatatgtttattaattcatgttttgtaatttatgggatagcgattttttttactgtctgtattttcttttttaattatgttttaattgtatttattttatttttattattgttctttttatagtattattttaaaacaaaatgtattttctaagaacttataataataataatataaattttaataaaaattatatttatcttttacaatatgaacataaagtacaacattaatatatagcttttaatatttttattcctaatcatgtaaatcttaaatttttctttttaaacatatgttaaatatttatttctcattatatataagaacatatttattacatctagaggtaccgagctcgttttcgacactggatggcggcgttagtatcgaatcgacagcagtatagcgaccagcattcacatacgattgacgcatgatattactttctgcgcacttaacttcgcatctgggcagatgatgtcgaggcgaaaaaaaatataaatcacgctaacatttgattaaaatagaacaactacaatataaaaaaactatacaaatgacaagttcttgaaaacaagaatctttttattgtcagtactgattagaaaaactcatcgagcatcaaatgaaactgcaatttattcatatcaggattatcaataccatatttttgaaaaagccgtttctgtaatgaaggagaaaactcaccgaggcagttccataggatggcaagatcctggtatcggtctgcgattccgactcgtccaacatcaatacaacctattaatttcccctcgtcaaaaataaggttatcaagtgagaaatcaccatgagtgacgactgaatccggtgagaatggcaaaagcttatgcatttctttccagacttgttcaacaggccagccattacgctcgtcatcaaaatcactcgcatcaaccaaaccgttattcattcgtgattgcgcctgagcgagacgaaatacgcgatcgctgttaaaaggacaattacaaacaggaatcgaatgcaaccggcgcaggaacactgccagcgcatcaacaatattttcacctgaatcaggatattcttctaatacctggaatgctgttttgccggggatcgcagtggtgagtaaccatgcatcatcaggagtacggataaaatgcttgatggtcggaagaggcataaattccgtcagccagtttagtctgaccatctcatctgtaacatcattggcaacgctacctttgccatgtttcagaaacaactctggcgcatcgggcttcccatacaatcgatagattgtcgcacctgattgcccgacattatcgcgagcccatttatacccatataaatcagcatccatgttggaatttaatcgcggcctcgaaacgtgagtcttttccttacccatggttgtttatgttcggatgtgatgtgagaactgtatcctagcaagattttaaaaggaagtatatgaaagaagaacctcagtggcaaatcctaaccttttatatttctctacaggggcgcggcgtggggacaattcaacgcgtctgtgaggggagcgtttccctgctcgcaggtctgcagcgaggagccgtaatttttgcttcgcgccgtgcggccatcaaaatgtatggatgcaaatgattatacatggggatgtatgggctaaatgtacgggcgacagtcacatcatgcccctgagctgcgcacgtcaagactgtcaaggagggtattctgggcctccatgtcgctggcctaacattagtaatgtaggtctgactttcactcatataagtcttatggtaactaaactaaggtcttacctttactgatatatgtcttactttcactaacttaggtattacttttactaacttaggtcttaaattcagtaactaaggtcatacttcgactaactaaggtcttacattcactgatataggtcttatgattactaacttaggtcctaatttgactaacataagtcctaacattagtaatgtaggtcttaacttaactaacttaggtcttaccttcactaatataggtcttaatattactgacttaagtaattaaggtactaacttaggtcgtaaggtaactaatatataggtcttaaggtaactaatttaggtcttgacttaataaatataggtcctaacataaatagtataggtcctaatataagtactataggccttaacttaaccaacataggtcctaacataagttatataggtcttaacgtaactaacataagtcattaaggtactaagtttggtcttaatttaacaataacatgtcgctggcctaacattagtaatgtaggtctgactttcactcatataagtcttatggtaactaaactaaggtcttacctttactgatatatgtcttactttcactaacttaggtattacttttactaacttaggtcttaaattcagtaactaaggtcatacttcgactaactaaggtcttacattcactgatataggtcttatgattactaacttaggtcctaatttgactaacataagtcctaacattagtaatgtaggtcttaacttaactaacttaggtcttaccttcactaatataggtcttaatattactgacttaagtaattaaggtactaacttaggtcgtaaggtaactaatatataggtcttaaggtaactaatttaggtcttgacttaataaatataggtcctaacataaatagtataggtcctaatataagtactataggccttaacttaaccaacataggtcctaacataagttatataggtcttaacgtaactaacataagtcattaaggtactaagtttggtcttaatttaacaataaccatgtcgctggccgggtggtcttaatttaacaaatatagaccatgtcgctggccgggtgacccggcggggacgaggcaagctaaacagatcctcgtgatacgcctatttttataggttaatgtcatgataataatggtttcttaggacggatcgcttgcctgtaacttacacgcgcctcgtatcttttaatgatggaataatttgggaatttactctgtgtttatttatttttatgttttgtatttggattttagaaagtaaataaagaaggtagaagagttacggaatgaagaaaaaaaaataaacaaaggtttaaaaaatttcaacaaaaagcgtactttacatatatatttattagacaagaaaagcagattaaatagatatacattcgattaacgataagtaaaatgtaaaatcacaggattttcgtgtgtggtcttctacacagacaagatgaaacaattcggcattaatacctgagagcaggaagagcaagataaaaggtagtatttgttggcgatccccctagagtcttttacatcttcggaaaacaaaaactattttttctttaatttctttttttactttctatttttaatttatatatttatattaaaaaatttaaattataattatttttatagcacgtgatgaaaaggacccaggtggcacttttcggggaaatctcgacctgcagcgtacgaagct

SEQ ID NO: 388 - DNA, 12044 bp, synthetic construct
  misc_feature 1..12044: note = Description of Artificial Sequence: Synthetic polynucleotide
  source 1..12044: mol_type = other DNA
gcctcactgattaagcattggtaactgtcagaccaagtttactcatatatactttagattgatttaaaacttcatttttaatttaaaaggatctaggtgaagatcctttttgataatctcatgaccaaaatcccttaacgtgagttttcgttccactgagcgtcagaccccgtagaaaagatcaaaggatcttcttgagatcctttttttctgcgcgtaatctgctgcttgcaaacaaaaaaaccaccgctaccagcggtggtttgtttgccggatcaagagctaccaactctttttccgaaggtaactggcttcagcagagcgcagataccaaatactgttcttctagtgtagccgtagttaggccaccacttcaagaactctgtagcaccgcctacatacctcgctctgctaatcctgttaccagtggctgctgccagtggcgataagtcgtgtcttaccgggttggactcaagacgatagttaccggataaggcgcagcggtcgggctgaacggggggttcgtgcacacagcccagcttggagcgaacgacctacaccgaactgagatacctacagcgtgagctatgagaaagcgccacgcttcccgaagggagaaaggcggacaggtatccggtaagcggcagggtcggaacaggagagcgcacgagggagcttccagggggaaacgcctggtatctttatagtcctgtcgggtttcgccacctctgacttgagcgtcgatttttgtgatgctcgtcaggggggcggagcctatggaaaaacgccagcaacgcggcctttttacggttcctggccttttgctggccttttgctcacatgttctttcctgcgttatcccctgattctgtggataaccgtattaccgcctttgagtgagctgataccgctcgccgcagccgaacgaccgagcgcagcgagtcagtgagcgaggaagcggaagagcgcccaatacgcaaaccgcctctccccgcgcgttggccgattcattaatgcagctggcacgacaggtttcccgactggaaagcgggcagtgagcgcaacgcaattaatgtgagttagctcactcattaggcaccccaggctttacactttatgcttccggctcgtatgttgtgtggaattgtgagcggataacaatttcacacaggaaacagctatgaccatgattacgccaagctatttaggtgacactatagaatactcaagcttggggggatcctctagagtcgactaatacgactcactataggaacataatctatagcggcgttttagagctagaaatagcaagttaaaataaggctagtccgttatcaacttgaaaaagtggcaccgagtcggtgctagcataaccccttggggcctctaaacgggtcttgaggggttttttggtcgacctgcaggcatgctatttgatgaattaactacacttaaaataatacaattattattaaatttttttttgatttatttattaatttttaaacttaatcatttgtatttgggaggaattatatatatctttataattattttatttttttttatttttttatttttttattattattatttttttttattttttttttttactgtatcaaagaaaaacctttaaaaaaaaaattataatttccccatcttactatatttttaatacatacgttttaaggaattaaattagacaaaagctatattatgctttacatataattagaatttataaacgtttggttattagatatttcatgtctcagtaaagtctttcaatacatatgtaaaaaaatatatatgaatacacataagttgttaatatattttatatgcataaatgtataaatatatatatatatatatatatatgtatgtatgtatatgtgtgtatatgaaattatttcaatgtttaattttttaaattttaatttttttttttttttttttttttattatgtatattgatctttattatttaaatattacttttttcgttttttcttctttttattatttttttttttttttatattttatacaaatggtaattcaaataaaaggtataaatttatatttaattttcttttatggataaataaaagaaaaatataaatatataaaaatataaaaatatatatatgtatattggggtgatgataaaatgaaagataatatatatatatatatatctttatttttttttttttgtagaccccattgtgagtacataaatatattatataactcgggagcatcagtcatggaattcttatttctttttcttttttgcctggccggcctttttcgtggccgccggccttttgtcgcctcccagctgagacaggtcgatccgtgtctcgtacaggccggtgatgctctggtggatcagggtggcgtccagcacctctttggtgctggtgtacctcttccggtcgatggtggtgtcaaagtacttgaaggcggcaggggctcccagattggtcagggtaaacaggtggatgatattctcggcctgctctctgatgggcttatcccggtgcttgttgtaggcggacagcactttgtccagattagcgtcggccaggatcactctcttggagaactcgctgatctgctcgatgatctcgtccaggtagtgcttgtgctgttccacaaacagctgtttctgctcattatcctcgggggagcccttcagcttctcatagtggctggccaggtacaggaagttcacatatttggagggcagggccagttcgtttcccttctgcagttcgccggcagaggccagcattctcttccggccgttttccagctcgaacagggagtacttaggcagcttgatgatcaggtcctttttcacttctttgtagcccttggcttccagaaagtcgatgggattcttctcgaagctgcttctttccatgatggtgatccccagcagctctttcacactcttcagtttcttggacttgcccttttccactttggccaccaccagcacagaataggccacggtggggctgtcgaagccgccgtacttcttagggtcccagtccttctttctggcgatcagcttatcgctgttcctcttgggcaggatagactctttgctgaagccgcctgtctgcacctcggtctttttcacgatattcacttggggcatgctcagcactttccgcacggtggcaaaatcccggcccttatcccacacgatctccccggtttcgccgtttgtctcgatcagaggccgcttccggatctcgccgttggccagggtaatctcggtcttgaaaaagttcatgatgttgctgtagaagaagtacttggcggtagccttgccgatttcctgctcgctcttggcgatcatcttccgcacgtcgtacaccttgtagtcgccgtacacgaactcgctttccagcttagggtactttttgatcagggcggttcccacgacggcgttcaggtaggcgtcgtgggcgtggtggtagttgttgatctcgcgcactttgtaaaactggaaatccttccggaaatcggacaccagcttggacttcagggtgatcactttcacttcccggatcagcttgtcattctcgtcgtacttagtgttcatccgggagtccaggatctgtgccacgtgctttgtgatctgccgggtttccaccagctgtctcttgatgaagccggccttatccagttcgctcaggccgcctctctcggccttggtcagattgtcgaactttctctgggtaatcagcttggcgttcagcagctgccgccagtagttcttcatcttcttcacgacctcttcggagggcacgttgtcgctcttgccccggttcttgtcgcttctggtcagcaccttgttgtcgatggagtcgtccttcagaaagctctgaggcacgatatggtccacatcgtagtcggacagccggttgatgtccagttcctggtccacgtacatatcccgcccattctgcaggtagtacaggtacagcttctcgttctgcagctgggtgttttccacggggtgttctttcaggatctggctgcccagctctttgatgccctcttcgatccgcttcattctctcgcggctgttcttctgtcccttctgggtggtctggttctctctggccatttcgatcacgatgttctcgggcttgtgccggcccatcactttcacgagctcgtccaccaccttcactgtctgcaggatgcccttcttaatggcggggctgccggccagattggcaatgtgctcgtgcaggctatcgccctggccggacacctgggctttctggatgtcctctttaaaggtcaggctgtcgtcgtggatcagctgcatgaagtttctgttggcgaagccgtcggacttcaggaaatccaggattgtcttgccggactgcttgtcccggatgccgttgatcagcttccggctcagcctgccccagccggtgtatctccgccgcttcagctgcttcatcactttgtcgtcgaacaggtgggcataggttttcagccgttcctcgatcatctctctgtcctcaaacagtgtcagggtcagcacgatatcttccagaatgtcctcgttttcctcattgtccaggaagtccttgtccttgataattttcagcagatcgtggtatgtgcccagggaggcgttgaaccgatcttccacgccggagatttccacggagtcgaagcactcgattttcttgaagtagtcctctttcagctgcttcacggtcactttccggttggtcttgaacagcaggtccacgatggcctttttctgctcgccgctcaggaaggcgggctttctcattccctcggtcacgtatttcactttggtcagctcgttatacacggtgaagtactcgtacagcaggctgtgcttgggcagcaccttctcgttgggcaggttcttatcgaagttggtcatccgctcgatgaagctctgggcggaagcgcccttgtccaccacttcctcgaagttccagggggtgatggtttcctcgctctttctggtcatccaggcgaatctgctgtttcccctggccagagggcccacgtagtaggggatgcggaaggtcaggatcttctcgatcttttcccggttgtccttcaggaatgggtaaaaatcttcctgccgccgcagaatggcgtgcagctctcccaggtggatctggtgggggatgctgccgttgtcgaaggtccgctgcttccgcagcaggtcctctctgttcagcttcacgagcagttcctcggtgccgtccatcttttccaggatgggcttgatgaacttgtagaactcttcctggctggctccgccgtcaatgtagccggcgtagccgttcttgctctggtcgaagaaaatctctttgtacttctcaggcagctgctgccgcacgagagctttcagcagggtcaggtcctggtggtgctcgtcgtatctcttgatcatagaggcgctcaggggggccttggtgatctcggtgttcactctcaggatgtcgctcagcaggatggcgtcggacaggttcttggcggccagaaacaggtcggcgtactggtcgccgatctgggccagcaggttgtccaggtcgtcgtcgtaggtgtccttgctcagctgcagtttggcatcctcggccaggtcgaagttgctcttgaagttgggggtcaggcccaggctcagggcaatcaggtttccgaacaggccattcttcttctcgccgggcagctgggcgatcagattttccagccgtctgctcttgctcagtctggcagacaggatggccttggcgtccacgccgctggcgttgatggggttttcctcgaacagctggttgtaggtctgcaccagctggatgaacagcttgtccacgtcgctgttgtcggggttcaggtcgccctcgatcaggaagtggccccggaacttgatcatgtgggccagggccagatagatcagccgcaggtcggccttgtcggtgctgtccaccagtttctttctcaggtggtagatggtggggtacttctcgtggtaggccacctcgtccacgatgttgccgaagatggggtgccgctcgtgcttcttatcctcttccaccaggaaggactcttccagtctgtggaagaagctgtcgtccaccttggccatctcgttgctgaagatctcttgcagatagcagatccggttcttccgtctggtgtatcttcttctggcggttctcttcagccgggtggcctcggctgtttcgccgctgtcgaacagcagggctccgatcaggttcttcttgatgctgtgccggtcggtgttgcccagcaccttgaatttcttgctgggcaccttgtactcgtcggtgatcacggcccagcccacagagttggtgccgatgtccaggccgatgctgtacttcttgtcggctgctgggactccgtggataccgaccttccgcttcttctttggggccatcttatcgtcatcgtctttgtaatcaatatcatgatccttgtagtctccgtcgtggtccttatagtccatttttctcgagggatcctgatatatttctattaggtatttattattataaaatataaatcttgaatgataataaataaaatattagttattccttttctagtttaaaatatacatattataaatatatatatatatatatatatttttattgtgacaagaatatataattataaattatattatttatttttgtatttttttttttttttttttttttttctttttttgttttatttttctttttttttataaatattatttttttcttttatcatgcacattggaataatacattaatatatatatatatattatattatacatatattgaataatgtttataaaaaatgcataacttatatgaatataattttttttaaatatgacaaaaagaaaaaaaaaaaaaaccaaaaaaaattaaaattgaaatgaaatatataaatatattatttatatatattatacattgtttaatactactacatgtatatatatatattatatatatatatatatatcaattttttcaaaaataaattaatataaaaagaggggaaaaaaaaaaaaaaaaaaaaaaaaagataattaagtaagcatttaaaaatatataaattgataatatataaaattaatcacatataaaagcttataaacactaggttagctaattcgcttgtaagaggtactctcgtttatgcaaaactatttgatatagcattttaacaagtacacatatatatatgtaatatatatactatatatatctattgcatgtgtactaagcatgtgcatggcatcccctttttctcgtgtttaaaacagtttgtatgataaaatataaaggatttgaaaaagagaaaaaaatatatgatctcatcctatatagcgccataatttttatttgggttgaataaaattttctactaaatttaggtgtaagtaaaataatggaatatatataagtacaataaaaaagtgcataaattaaaaaatttttataataaatattttttttaaaaaagtcaataataatattaaatatatataacacaggattatatatgttcactacaattttttatattataatataaattcttttcaattttcattttattttacatacactttccttttttgtcactatattttaatattcacatatttagtttaaatactggctatttctttctacatttgctagtaacaattgtgtagtgcttaaatatatacacacacctaaaacttacaaagtatcctaggaccatggccaagcctttgtctcaagaagaatccaccctcattgaaagagcaacggctacaatcaacagcatccccatctctgaagactacagcgtcgccagcgcagctctctctagcgacggccgcatcttcactggtgtcaatgtatatcattttactgggggaccttgtgcagaactcgtggtgctgggcactgctgctgctgcggcagctggcaacctgacttgtatcgtcgcgatcggaaatgagaacaggggcatcttgagcccctgcggacggtgccgacaggtgcttctcgatctgcatcctgggatcaaagccatagtgaaggacagtgatggacagccgacggcagttgggattcgtgaattgctgccctctggttatgtgtgggagggctaaccgcgggtaccccattaaatttatttaataatagattaaaaatattataaaaataaaaacataaacacagaaattacaaaaaaaatacatatgaattttttttttgtaatcttccttataaatatagaataatgaatcatataaaacatatcattattcatttatttacatttaaaattattgtttcagtatctttaatttattatgtatatataaaaataacttacaattttattaataaacaatatatgtttattaattcatgttttgtaatttatgggatagcgattttttttactgtctgtattttcttttttaattatgttttaattgtatttattttatttttattattgttctttttatagtattattttaaaacaaaatgtattttctaagaacttataataataataatataaattttaataaaaattatatttatcttttacaatatgaacataaagtacaacattaatatatagcttttaatatttttattcctaatcatgtaaatcttaaatttttctttttaaacatatgttaaatatttatttctcattatatataagaacatatttattacatctagaggtaccgagctcgttttcgacactggatggcggcgttagtatcgaatcgacagcagtatagcgaccagcattcacatacgattgacgcatgatattactttctgcgcacttaacttcgcatctgggcagatgatgtcgaggcgaaaaaaaatataaatcacgctaacatttgattaaaatagaacaactacaatataaaaaaactatacaaatgacaagttcttgaaaacaagaatctttttattgtcagtactgattagaaaaactcatcgagcatcaaatgaaactgcaatttattcatatcaggattatcaataccatatttttgaaaaagccgtttctgtaatgaaggagaaaactcaccgaggcagttccataggatggcaagatcctggtatcggtctgcgattccgactcgtccaacatcaatacaacctattaatttcccctcgtcaaaaataaggttatcaagtgagaaatcaccatgagtgacgactgaatccggtgagaatggcaaaagcttatgcatttctttccagacttgttcaacaggccagccattacgctcgtcatcaaaatcactcgcatcaaccaaaccgttattcattcgtgattgcgcctgagcgagacgaaatacgcgatcgctgttaaaaggacaattacaaacaggaatcgaatgcaaccggcgcaggaacactgccagcgcatcaacaatattttcacctgaatcaggatattcttctaatacctggaatgctgttttgccggggatcgcagtggtgagtaaccatgcatcatcaggagtacggataaaatgcttgatggtcggaagaggcataaattccgtcagccagtttagtctgaccatctcatctgtaacatcattggcaacgctacctttgccatgtttcagaaacaactctggcgcatcgggcttcccatacaatcgatagattgtcgcacctgattgcccgacattatcgcgagcccatttatacccatataaatcagcatccatgttggaatttaatcgcggcctcgaaacgtgagtcttttccttacccatggttgtttatgttcggatgtgatgtgagaactgtatcctagcaagattttaaaaggaagtatatgaaagaagaacctcagtggcaaatcctaaccttttatatttctctacaggggcgcggcgtggggacaattcaacgcgtctgtgaggggagcgtttccctgctcgcaggtctgcagcgaggagccgtaatttttgcttcgcgccgtgcggccatcaaaatgtatggatgcaaatgattatacatggggatgtatgggctaaatgtacgggcgacagtcacatcatgcccctgagctgcgcacgtcaagactgtcaaggagggtattctgggcctccatgtcgctggcctaacattagtaatgtaggtctgactttcactcatataagtcttatggtaactaaactaaggtcttacctttactgatatatgtcttactttcactaacttaggtattacttttactaacttaggtcttaaattcagtaactaaggtcatacttcgactaactaaggtcttacattcactgatataggtcttatgattactaacttaggtcctaatttgactaacataagtcctaacattagtaatgtaggtcttaacttaactaacttaggtcttaccttcactaatataggtcttaatattactgacttaagtaattaaggtactaacttaggtcgtaaggtaactaatatataggtcttaaggtaactaatttaggtcttgacttaataaatataggtcctaacataaatagtataggtcctaatataagtactataggccttaacttaaccaacataggtcctaacataagttatataggtcttaacgtaactaacataagtcattaaggtactaagtttggtcttaatttaacaataacatgtcgctggcctaacattagtaatgtaggtctgactttcactcatataagtcttatggtaactaaactaaggtcttacctttactgatatatgtcttactttcactaacttaggtattacttttactaacttaggtcttaaattcagtaactaaggtcatacttcgactaactaaggtcttacattcactgatataggtcttatgattactaacttaggtcctaatttgactaacataagtcctaacattagtaatgtaggtcttaacttaactaacttaggtcttaccttcactaatataggtcttaatattactgacttaagtaattaaggtactaacttaggtcgtaaggtaactaatatataggtcttaaggtaactaatttaggtcttgacttaataaatataggtcctaacataaatagtataggtcctaatataagtactataggccttaacttaaccaacataggtcctaacataagttatataggtcttaacgtaactaacataagtcattaaggtactaagtttggtcttaatttaacaataaccatgtcgctggccgggtggtcttaatttaacaaatatagaccatgtcgctggccgggtgacccggcggggacgaggcaagctaaacagatcctcgtgatacgcctatttttataggttaatgtcatgataataatggtttcttaggacggatcgcttgcctgtaacttacacgcgcctcgtatcttttaatgatggaataatttgggaatttactctgtgtttatttatttttatgttttgtatttggattttagaaagtaaataaagaaggtagaagagttacggaatgaagaaaaaaaaataaacaaaggtttaaaaaatttcaacaaaaagcgtactttacatatatatttattagacaagaaaagcagattaaatagatatacattcgattaacgataagtaaaatgtaaaatcacaggattttcgtgtgtggtcttctacacagacaagatgaaacaattcggcattaatacctgagagcaggaagagcaagataaaaggtagtatttgttggcgatccccctagagtcttttacatcttcggaaaacaaaaactattttttctttaatttctttttttactttctatttttaatttatatatttatattaaaaaatttaaattataattatttttatagcacgtgatgaaaaggacccaggtggcacttttcggggaaatctcgacctgcagcgtacgaagct

SEQ ID NO: 389 - DNA, 12044 bp, synthetic construct
  misc_feature 1..12044: note = Description of Artificial Sequence: Synthetic polynucleotide
  source 1..12044: mol_type = other DNA
gcctcactgattaagcattggtaactgtcagaccaagtttactcatatatactttagattgatttaaaacttcatttttaatttaaaaggatctaggtgaagatcctttttgataatctcatgaccaaaatcccttaacgtgagttttcgttccactgagcgtcagaccccgtagaaaagatcaaaggatcttcttgagatcctttttttctgcgcgtaatctgctgcttgcaaacaaaaaaaccaccgctaccagcggtggtttgtttgccggatcaagagctaccaactctttttccgaaggtaactggcttcagcagagcgcagataccaaatactgttcttctagtgtagccgtagttaggccaccacttcaagaactctgtagcaccgcctacatacctcgctctgctaatcctgttaccagtggctgctgccagtggcgataagtcgtgtcttaccgggttggactcaagacgatagttaccggataaggcgcagcggtcgggctgaacggggggttcgtgcacacagcccagcttggagcgaacgacctacaccgaactgagatacctacagcgtgagctatgagaaagcgccacgcttcccgaagggagaaaggcggacaggtatccggtaagcggcagggtcggaacaggagagcgcacgagggagcttccagggggaaacgcctggtatctttatagtcctgtcgggtttcgccacctctgacttgagcgtcgatttttgtgatgctcgtcaggggggcggagcctatggaaaaacgccagcaacgcggcctttttacggttcctggccttttgctggccttttgctcacatgttctttcctgcgttatcccctgattctgtggataaccgtattaccgcctttgagtgagctgataccgctcgccgcagccgaacgaccgagcgcagcgagtcagtgagcgaggaagcggaagagcgcccaatacgcaaaccgcctctccccgcgcgttggccgattcattaatgcagctggcacgacaggtttcccgactggaaagcgggcagtgagcgcaacgcaattaatgtgagttagctcactcattaggcaccccaggctttacactttatgcttccggctcgtatgttgtgtggaattgtgagcggataacaatttcacacaggaaacagctatgaccatgattacgccaagctatttaggtgacactatagaatactcaagcttggggggatcctctagagtcgactaatacgactcactataggaaatgatatggattttgggttttagagctagaaatagcaagttaaaataaggctagtccgttatcaacttgaaaaagtggcaccgagtcggtgctagcataaccccttggggcctctaaacgggtcttgaggggttttttggtcgacctgcaggcatgctatttgatgaattaactacacttaaaataatacaattattattaaatttttttttgatttatttattaatttttaaacttaatcatttgtatttgggaggaattatatatatctttataattattttatttttttttatttttttatttttttattattattatttttttttattttttttttttactgtatcaaagaaaaacctttaaaaaaaaaattataatttccccatcttactatatttttaatacatacgttttaaggaattaaattagacaaaagctatattatgctttacatataattagaatttataaacgtttggttattagatatttcatgtctcagtaaagtctttcaatacatatgtaaaaaaatatatatgaatacacataagttgttaatatattttatatgcataaatgtataaatatatatatatatatatatatatgtatgtatgtatatgtgtgtatatgaaattatttcaatgtttaattttttaaattttaatttttttttttttttttttttttattatgtatattgatctttattatttaaatattacttttttcgttttttcttctttttattatttttttttttttttatattttatacaaatggtaattcaaataaaaggtataaatttatatttaattttcttttatggataaataaaagaaaaatataaatatataaaaatataaaaatatatatatgtatattggggtgatgataaaatgaaagataatatatatatatatatatctttatttttttttttttgtagaccccattgtgagtacataaatatattatataactcgggagcatcagtcatggaattcttatttctttttcttttttgcctggccggcctttttcgtggccgccggccttttgtcgcctcccagctgagacaggtcgatccgtgtctcgtacaggccggtgatgctctggtggatcagggtggcgtccagcacctctttggtgctggtgtacctcttccggtcgatggtggtgtcaaagtacttgaaggcggcaggggctcccagattggtcagggtaaacaggtggatgatattctcggcctgctctctgatgggcttatcccggtgcttgttgtaggcggacagcactttgtccagattagcgtcggccaggatcactctcttggagaactcgctgatctgctcgatgatctcgtccaggtagtgcttgtgctgttccacaaacagctgtttctgctcattatcctcgggggagcccttcagcttctcatagtggctggccaggtacaggaagttcacatatttggagggcagggccagttcgtttcccttctgcagttcgccggcagaggccagcattctcttccggccgttttccagctcgaacagggagtacttaggcagcttgatgatcaggtcctttttcacttctttgtagcccttggcttccagaaagtcgatgggattcttctcgaagctgcttctttccatgatggtgatccccagcagctctttcacactcttcagtttcttggacttgcccttttccactttggccaccaccagcacagaataggccacggtggggctgtcgaagccgccgtacttcttagggtcccagtccttctttctggcgatcagcttatcgctgttcctcttgggcaggatagactctttgctgaagccgcctgtctgcacctcggtctttttcacgatattcacttggggcatgctcagcactttccgcacggtggcaaaatcccggcccttatcccacacgatctccccggtttcgccgtttgtctcgatcagaggccgcttccggatctcgccgttggccagggtaatctcggtcttgaaaaagttcatgatgttgctgtagaagaagtacttggcggtagccttgccgatttcctgctcgctcttggcgatcatcttccgcacgtcgtacaccttgtagtcgccgtacacgaactcgctttccagcttagggtactttttgatcagggcggttcccacgacggcgttcaggtaggcgtcgtgggcgtggtggtagttgttgatctcgcgcactttgtaaaactggaaatccttccggaaatcggacaccagcttggacttcagggtgatcactttcacttcccggatcagcttgtcattctcgtcgtacttagtgttcatccgggagtccaggatctgtgccacgtgctttgtgatctgccgggtttccaccagctgtctcttgatgaagccggccttatccagttcgctcaggccgcctctctcggccttggtcagattgtcgaactttctctgggtaatcagcttggcgttcagcagctgccgccagtagttcttcatcttcttcacgacctcttcggagggcacgttgtcgctcttgccccggttcttgtcgcttctggtcagcaccttgttgtcgatggagtcgtccttcagaaagctctgaggcacgatatggtccacatcgtagtcggacagccggttgatgtccagttcctggtccacgtacatatcccgcccattctgcaggtagtacaggtacagcttctcgttctgcagctgggtgttttccacggggtgttctttcaggatctggctgcccagctctttgatgccctcttcgatccgcttcattctctcgcggctgttcttctgtcccttctgggtggtctggttctctctggccatttcgatcacgatgttctcgggcttgtgccggcccatcactttcacgagctcgtccaccaccttcactgtctgcaggatgcccttcttaatggcggggctgccggccagattggcaatgtgctcgtgcaggctatcgccctggccggacacctgggctttctggatgtcctctttaaaggtcaggctgtcgtcgtggatcagctgcatgaagtttctgttggcgaagccgtcggacttcaggaaatccaggattgtcttgccggactgcttgtcccggatgccgttgatcagcttccggctcagcctgccccagccggtgtatctccgccgcttcagctgcttcatcactttgtcgtcgaacaggtgggcataggttttcagccgttcctcgatcatctctctgtcctcaaacagtgtcagggtcagcacgatatcttccagaatgtcctcgttttcctcattgtccaggaagtccttgtccttgataattttcagcagatcgtggtatgtgcccagggaggcgttgaaccgatcttccacgccggagatttccacggagtcgaagcactcgattttcttgaagtagtcctctttcagctgcttcacggtcactttccggttggtcttgaacagcaggtccacgatggcctttttctgctcgccgctcaggaaggcgggctttctcattccctcggtcacgtatttcactttggtcagctcgttatacacggtgaagtactcgtacagcaggctgtgcttgggcagcaccttctcgttgggcaggttcttatcgaagttggtcatccgctcgatgaagctctgggcggaagcgcccttgtccaccacttcctcgaagttccagggggtgatggtttcctcgctctttctggtcatccaggcgaatctgctgtttcccctggccagagggcccacgtagtaggggatgcggaaggtcaggatcttctcgatcttttcccggttgtccttcaggaatgggtaaaaatcttcctgccgccgcagaatggcgtgcagctctcccaggtggatctggtgggggatgctgccgttgtcgaaggtccgctgcttccgcagcaggtcctctctgttcagcttcacgagcagttcctcggtgccgtccatcttttccaggatgggcttgatgaacttgtagaactcttcctggctggctccgccgtcaatgtagccggcgtagccgttcttgctctggtcgaagaaaatctctttgtacttctcaggcagctgctgccgcacgagagctttcagcagggtcaggtcctggtggtgctcgtcgtatctcttgatcatagaggcgctcaggggggccttggtgatctcggtgttcactctcaggatgtcgctcagcaggatggcgtcggacaggttcttggcggccagaaacaggtcggcgtactggtcgccgatctgggccagcaggttgtccaggtcgtcgtcgtaggtgtccttgctcagctgcagtttggcatcctcggccaggtcgaagttgctcttgaagttgggggtcaggcccaggctcagggcaatcaggtttccgaacaggccattcttcttctcgccgggcagctgggcgatcagattttccagccgtctgctcttgctcagtctggcagacaggatggccttggcgtccacgccgctggcgttgatggggttttcctcgaacagctggttgtaggtctgcaccagctggatgaacagcttgtccacgtcgctgttgtcggggttcaggtcgccctcgatcaggaagtggccccggaacttgatcatgtgggccagggccagatagatcagccgcaggtcggccttgtcggtgctgtccaccagtttctttctcaggtggtagatggtggggtacttctcgtggtaggccacctcgtccacgatgttgccgaagatggggtgccgctcgtgcttcttatcctcttccaccaggaaggactcttccagtctgtggaagaagctgtcgtccaccttggccatctcgttgctgaagatctcttgcagatagcagatccggttcttccgtctggtgtatcttcttctggcggttctcttcagccgggtggcctcggctgtttcgccgctgtcgaacagcagggctccgatcaggttcttcttgatgctgtgccggtcggtgttgcccagcaccttgaatttcttgctgggcaccttgtactcgtcggtgatcacggcccagcccacagagttggtgccgatgtccaggccgatgctgtacttcttgtcggctgctgggactccgtggataccgaccttccgcttcttctttggggccatcttatcgtcatcgtctttgtaatcaatatcatgatccttgtagtctccgtcgtggtccttatagtccatttttctcgagggatcctgatatatttctattaggtatttattattataaaatataaatcttgaatgataataaataaaatattagttattccttttctagtttaaaatatacatattataaatatatatatatatatatatatttttattgtgacaagaatatataattataaattatattatttatttttgtatttttttttttttttttttttttttctttttttgttttatttttctttttttttataaatattatttttttcttttatcatgcacattggaataatacattaatatatatatatatattatattatacatatattgaataatgtttataaaaaatgcataacttatatgaatataattttttttaaatatgacaaaaagaaaaaaaaaaaaaaccaaaaaaaattaaaattgaaatgaaatatataaatatattatttatatatattatacattgtttaatactactacatgtatatatatatattatatatatatatatatatcaattttttcaaaaataaattaatataaaaagaggggaaaaaaaaaaaaaaaaaaaaaaaaagataattaagtaagcatttaaaaatatataaattgataatatataaaattaatcacatataaaagcttataaacactaggttagctaattcgcttgtaagaggtactctcgtttatgcaaaactatttgatatagcattttaacaagtacacatatatatatgtaatatatatactatatatatctattgcatgtgtactaagcatgtgcatggcatcccctttttctcgtgtttaaaacagtttgtatgataaaatataaaggatttgaaaaagagaaaaaaatatatgatctcatcctatatagcgccataatttttatttgggttgaataaaattttctactaaatttaggtgtaagtaaaataatggaatatatataagtacaataaaaaagtgcataaattaaaaaatttttataataaatattttttttaaaaaagtcaataataatattaaatatatataacacaggattatatatgttcactacaattttttatattataatataaattcttttcaattttcattttattttacatacactttccttttttgtcactatattttaatattcacatatttagtttaaatactggctatttctttctacatttgctagtaacaattgtgtagtgcttaaatatatacacacacctaaaacttacaaagtatcctaggaccatggccaagcctttgtctcaagaagaatccaccctcattgaaagagcaacggctacaatcaacagcatccccatctctgaagactacagcgtcgccagcgcagctctctctagcgacggccgcatcttcactggtgtcaatgtatatcattttactgggggaccttgtgcagaactcgtggtgctgggcactgctgctgctgcggcagctggcaacctgacttgtatcgtcgcgatcggaaatgagaacaggggcatcttgagcccctgcggacggtgccgacaggtgcttctcgatctgcatcctgggatcaaagccatagtgaaggacagtgatggacagccgacggcagttgggattcgtgaattgctgccctctggttatgtgtgggagggctaaccgcgggtaccccattaaatttatttaataatagattaaaaatattataaaaataaaaacataaacacagaaattacaaaaaaaatacatatgaattttttttttgtaatcttccttataaatatagaataatgaatcatataaaacatatcattattcatttatttacatttaaaattattgtttcagtatctttaatttattatgtatatataaaaataacttacaattttattaataaacaatatatgtttattaattcatgttttgtaatttatgggatagcgattttttttactgtctgtattttcttttttaattatgttttaattgtatttattttatttttattattgttctttttatagtattattttaaaacaaaatgtattttctaagaacttataataataataatataaattttaataaaaattatatttatcttttacaatatgaacataaagtacaacattaatatatagcttttaatatttttattcctaatcatgtaaatcttaaatttttctttttaaacatatgttaaatatttatttctcattatatataagaacatatttattacatctagaggtaccgagctcgttttcgacactggatggcggcgttagtatcgaatcgacagcagtatagcgaccagcattcacatacgattgacgcatgatattactttctgcgcacttaacttcgcatctgggcagatgatgtcgaggcgaaaaaaaatataaatcacgctaacatttgattaaaatagaacaactacaatataaaaaaactatacaaatgacaagttcttgaaaacaagaatctttttattgtcagtactgattagaaaaactcatcgagcatcaaatgaaactgcaatttattcatatcaggattatcaataccatatttttgaaaaagccgtttctgtaatgaaggagaaaactcaccgaggcagttccataggatggcaagatcctggtatcggtctgcgattccgactcgtccaacatcaatacaacctattaatttcccctcgtcaaaaataaggttatcaagtgagaaatcaccatgagtgacgactgaatccggtgagaatggcaaaagcttatgcatttctttccagacttgttcaacaggccagccattacgctcgtcatcaaaatcactcgcatcaaccaaaccgttattcattcgtgattgcgcctgagcgagacgaaatacgcgatcgctgttaaaaggacaattacaaacaggaatcgaatgcaaccggcgcaggaacactgccagcgcatcaacaatattttcacctgaatcaggatattcttctaatacctggaatgctgttttgccggggatcgcagtggtgagtaaccatgcatcatcaggagtacggataaaatgcttgatggtcggaagaggcataaattccgtcagccagtttagtctgaccatctcatctgtaacatcattggcaacgctacctttgccatgtttcagaaacaactctggcgcatcgggcttcccatacaatcgatagattgtcgcacctgattgcccgacattatcgcgagcccatttatacccatataaatcagcatccatgttggaatttaatcgcggcctcgaaacgtgagtcttttccttacccatggttgtttatgttcggatgtgatgtgagaactgtatcctagcaagattttaaaaggaagtatatgaaagaagaacctcagtggcaaatcctaaccttttatatttctctacaggggcgcggcgtggggacaattcaacgcgtctgtgaggggagcgtttccctgctcgcaggtctgcagcgaggagccgtaatttttgcttcgcgccgtgcggccatcaaaatgtatggatgcaaatgattatacatggggatgtatgggctaaatgtacgggcgacagtcacatcatgcccctgagctgcgcacgtcaagactgtcaaggagggtattctgggcctccatgtcgctggcctaacattagtaatgtaggtctgactttcactcatataagtcttatggtaactaaactaaggtcttacctttactgatatatgtcttactttcactaacttaggtattacttttactaacttaggtcttaaattcagtaactaaggtcatacttcgactaactaaggtcttacattcactgatataggtcttatgattactaacttaggtcctaatttgactaacataagtcctaacattagtaatgtaggtcttaacttaactaacttaggtcttaccttcactaatataggtcttaatattactgacttaagtaattaaggtactaacttaggtcgtaaggtaactaatatataggtcttaaggtaactaatttaggtcttgacttaataaatataggtcctaacataaatagtataggtcctaatataagtactataggccttaacttaaccaacataggtcctaacataagttatataggtcttaacgtaactaacataagtcattaaggtactaagtttggtcttaatttaacaataacatgtcgctggcctaacattagtaatgtaggtctgactttcactcatataagtcttatggtaactaaactaaggtcttacctttactgatatatgtcttactttcactaacttaggtattacttttactaacttaggtcttaaattcagtaactaaggtcatacttcgactaactaaggtcttacattcactgatataggtcttatgattactaacttaggtcctaatttgactaacataagtcctaacattagtaatgtaggtcttaacttaactaacttaggtcttaccttcactaatataggtcttaatattactgacttaagtaattaaggtactaacttaggtcgtaaggtaactaatatataggtcttaaggtaactaatttaggtcttgacttaataaatataggtcctaacataaatagtataggtcctaatataagtactataggccttaacttaaccaacataggtcctaacataagttatataggtcttaacgtaactaacataagtcattaaggtactaagtttggtcttaatttaacaataaccatgtcgctggccgggtggtcttaatttaacaaatatagaccatgtcgctggccgggtgacccggcggggacgaggcaagctaaacagatcctcgtgatacgcctatttttataggttaatgtcatgataataatggtttcttaggacggatcgcttgcctgtaacttacacgcgcctcgtatcttttaatgatggaataatttgggaatttactctgtgtttatttatttttatgttttgtatttggattttagaaagtaaataaagaaggtagaagagttacggaatgaagaaaaaaaaataaacaaaggtttaaaaaatttcaacaaaaagcgtactttacatatatatttattagacaagaaaagcagattaaatagatatacattcgattaacgataagtaaaatgtaaaatcacaggattttcgtgtgtggtcttctacacagacaagatgaaacaattcggcattaatacctgagagcaggaagagcaagataaaaggtagtatttgttggcgatccccctagagtcttttacatcttcggaaaacaaaaactattttttctttaatttctttttttactttctatttttaatttatatatttatattaaaaaatttaaattataattatttttatagcacgtgatgaaaaggacccaggtggcacttttcggggaaatctcgacctgcagcgtacgaagct